European Patent Specification EP 3 498 850 B1, published February 19, 2025. Title: HETEROLOGOUS EXPRESSION CASSETTE, DNA CONSTRUCT, AND VACCINE COMPOSITION FOR IMMUNIZING AGAINST FLAVIVIRUS AND/OR OTHER PATHOGENS. Applicant: Fundacao Oswaldo Cruz. The sequence listing filed with the application follows.

SEQUENCE LISTING (72 sequences)

SEQ ID NO: 1 - DNA, 11800 bp, Yellow fever virus
agtaaatcctgtgtgctaattgaggtgcattggtctgcaaatcgagttgctaggcaataaacacatttggattaattttaatcgttcgttgagcgattagcagagaactgaccagaacatgtctggtcgtaaagctcagggaaaaaccctgggcgtcaatatggtacgacgaggagttcgctccttgtcaaacaaaataaaacaaaaaacaaaacaaattggaaacagacctggaccttcaagaggtgttcaaggatttatctttttctttttgttcaacattttgactggaaaaaagatcacagcccacctaaagaggttgtggaaaatgctggacccaagacaaggcttggctgttctaaggaaagtcaagagagtggtggccagtttgatgagaggattgtcctcaaggaaacgccgttcccatgatgttctgactgtgcaattcctaattttgggaatgctgttgatgaccggtggagtgaccttggtgcggaaaaacagatggttgctcctaaatgtgacatctgaggacctcgggaaaacattctctgtgggcacaggcaactgcacaacaaacattttggaagccaagtactggtgcccagactcaatggaatacaactgtcccaatctcagtccaagagaggagccagatgacattgattgctggtgctatggggtggaaaacgttagagtcgcatatggtaagtgtgactcagcaggcaggtctaggaggtcaagaagggccattgacttgcctacgcatgaaaaccatggtttgaagacccggcaagaaaaatggatgactggaagaatgggtgaaaggcaactccaaaagattgagagatggttcgtgaggaaccccttttttgcagtgacggctctgaccattgcctaccttgtgggaagcaacatgacgcaacgagtcgtgattgccctactggtcttggctgttggtccggcctactcagctcactgcattggaattactgacagggatttcattgagggggtgcatggaggaacttgggtttcagctaccctggagcaagacaagtgtgtcactgttatggcccctgacaagccttcattggacatctcactagagacagtagccattgatagacctgctgaggcgaggaaagtgtgttacaatgcagttctcactcatgtgaagattaatgacaagtgccccagcactggagaggcccacctagctgaagagaacgaaggggacaatgcgtgcaagcgcacttattctgatagaggctggggcaatggctgtggcctatttgggaaagggagcattgtggcatgcgccaaattcacttgtgccaaatccatgagtttgtttgaggttgatcagaccaaaattcagtatgtcatcagagcacaattgcatgtaggggccaagcaggaaaattggaataccagcattaagactctcaagtttgatgccctgtcaggctcccaggaagtcgagttcattgggtatggaaaagctacactggaatgccaggtgcaaactgcggtggactttggtaacagttacatcgctgagatggaaacagagagctggatagtggacagacagtgggcccaggacttgaccctgccatggcagagtggaagtggcggggtgtggagagagatgcatcatcttgtcgaatttgaacctccgcatgccgccactatcagagtactggccctgggaaaccaggaaggctccttgaaaacagctcttactggcgcaatgagggttacaaaggacacaaatgacaacaacctttacaaactacatggtggacatgtttcttgcagagtgaaattgtcagctttgacactcaaggggacatcctacaaaatatgcactgacaaaatgttttttgtcaagaacccaactgacactggccatggcactgttgtgatgcaggtgaaagtgtcaaaaggagccccctgcaggattccagtgatagtagctgatgatcttacagcggcaatcaataaaggcattttggttacagttaaccccatcgcctcaaccaatgatgatgaagtgctgattgaggtgaacccaccttttggagacagctacattatcgttgggagaggagattcacgtctcacttaccagtggcacaaagagggaagctcaataggaaagttgttcactcagaccatgaaaggcgtggaacgcctggccgtcatgggagacaccgcctgggatttcagctccgctggagggttcttcacttcggttgggaaaggaattcatacggtgtttggctctgcctttcaggggctatttggcggcttgaactggataacaaaggtcatcatgggggcggtacttatatgggttggcatcaacacaagaaacatgacaatgtccatgagcatgatcttggtaggagtgatcatgatgtttttgtctctaggagttggggcggatcaaggatgcgccatcaactttggcgtgagcaagggcgaggagctgttcaccggggtggtgcccatcctggtcgagctggacggcgacgtaaacggccacaagttcagcgtgtccggcgagggcgagggcgatgccacctacggcaagctgaccctgaagttcatctgcaccaccggcaagctgcccgtgccctggcccaccctcgtgaccaccctgacctacggcgtgcagtgcttcagccgctaccccgaccacatgaagcagcacgacttcttcaagtccgccatgcccgaaggctacgtccaggagcgcaccatcttcttcaaggacgacggcaactacaagacccgcgccgaggtgaagttcgagggcgacaccctggtgaaccgcatcgagctgaagggcatcgacttcaaggaggacggcaacatcctggggcacaagctggagtacaactacaacagccacaacgtctatatcatggccgacaagcagaagaacggcatcaaggtgaacttcaagatccgccacaacatcgaggacggcagcgtgcagctcgccgaccactaccagcagaacacccccatcggcgacggccccgtgctgctgcccgacaaccactacctgagcacccagtccgccctgagcaaagaccccaacgagaagcgcgatcacatggtcctgctggagttcgtgaccgccgccgggatcactctcggcatggacgagctgtacaagacatcattgggaaaggctgtgcaccaggtttttggaagtgtgtatacaaccatgtttggaggagtctcatggatgattagaatcctaattgggttcttagtgttgtggattggcacgaactcgaggaacacttcaatggctatgacgtgcatagctgttggaggaatcactctgtttctgggcttcacagttggcgccgatcaaggatgcgccatcaactttggcaagagagagctcaagtgcggagatggtatcttcatatttagagactctgatgactggctgaacaagtactcatactatccagaagatcctgtgaagcttgcatcaatagtgaaagcctcttttgaagaagggaagtgtggcctaaattcagttgactcccttgagcatgagatgtggagaagcagggcagatgagatcaatgccatttttgaggaaaacgaggtggacatttctgttgtcgtgcaggatccaaagaatgtttaccagagaggaactcatccattttccagaattcgggatggtctgcagtatggttggaagacttggggtaagaaccttgtgttctccccagggaggaagaatggaagcttcatcatagatggaaagtccaggaaagaatgcccgttttcaaaccgggtctggaattctttccagatagaggagtttgggacgggagtgttcaccacacgcgtgtacatggacgcagtctttgaatacaccatagactgcgatggatctatcttgggtgcagcggtgaacggaaaaaagagtgcccatggctctccaacattttggatgggaagtcatgaagtaaatgggacatggatgatccacaccttggaggcattagattacaaggagtgtgagtggccactgacacatacgattggaacatcagttgaagagagtgaaatgttcatgccgagatcaatcggaggcccagttagctctcacaatcatatccctggatacaaggttcagacgaacggaccttggatgcaggtaccactagaagtgaagagagaagcttgcccagggactagcgtgatcattgatggcaactgtgatggacggggaaaatcaaccagatccaccacggatagcgggaaagttattcctgaatggtgttgccgctcctgcacaatgccgcctgtgagcttccatggtagtgatgggtgttggtatcccatggaaattaggccaaggaaaacgcatgaaagccatctggtgcgctcctgggttacagctggagaaatacatgctgtcccttttggtttggtgagcatgatgatagcaatggaagtggtcctaaggaaaagacagggaccaaagcaaatgttggttggaggagtagtgctcttgggagcaatgctggtcgggcaagtaactctccttgatttgctgaaactcacagtggctgtgggattgcatttccatgagatgaacaatggaggagacgccatgtatatggcgttgattgctgccttttcaatcagaccagggctgctcatcggctttgggctcaggaccctatggagccctcgggaacgccttgtgctgaccctaggagcagccatggtggagattgccttgggtggcgtgatgggcggcctgtggaagtatctaaatgcagtttctctctgcatcctgacaataaatgctgttgcttctaggaaagcatcaaataccatcttgcccctcatggctctgttgacacctgtcactatggctgaggtgagacttgccgcaatgttcttttgtgccatggttatcataggggtccttcaccagaatttcaaggacacctccatgcagaagactatacctctggtggccctcacactcacatcttacctgggcttgacacaaccttttttgggcctgtgtgcatttctggcaacccgcatatttgggcgaaggagtatcccagtgaatgaggcactcgcagcagctggtctagtgggagtgctggcaggactggcttttcaggagatggagaacttccttggtccgattgcagttggaggactcctgatgatgctggttagcgtggctgggagggtggatgggctagagctcaagaagcttggtgaagtttcatgggaagaggaggcggagatcagcgggagttccgcccgctatgatgtggcactcagtgaacaaggggagttcaagctgctttctgaagagaaagtgccatgggaccaggttgtgatgacctcgctggccttggttggggctgccctccatccatttgctcttctgctggtccttgctgggtggctgtttcatgtcaggggagctaggagaagtggggatgtcttgtgggatattcccactcctaagatcatcgaggaatgtgaacatctggaggatgggatttatggcatattccagtcaaccttcttgggggcctcccagcgaggagtgggagtggcacagggaggggtgttccacacaatgtggcatgtcacaagaggagctttccttgtcaggaatggcaagaagttgattccatcttgggcttcagtaaaggaagaccttgtcgcctatggtggctcatggaagttggaaggcagatgggatggagaggaagaggtccagttgatcgcggctgttccaggaaagaacgtggtcaacgtccagacaaaaccgagcttgttcaaagtgaggaatgggggagaaatcggggctgtcgctcttgactatccgagtggcacttcaggatctcctattgttaacaggaacggagaggtgattgggctgtacggcaatggcatccttgtcggtgacaactccttcgtgtccgccatatcccagactgaggtgaaggaagaaggaaaggaggagctccaagagatcccgacaatgctaaagaaaggaatgacaactgtccttgattttcatcctggagctgggaagacaagacgtttcctcccacagatcttggccgagtgcgcacggagacgcttgcgcactcttgtgttggcccccaccagggttgttctttctgaaatgaaggaggcttttcacggcctggacgtgaaattccacacacaggctttttccgctcacggcagcgggagagaagtcattgatgccatgtgccatgccaccctaacttacaggatgttggaaccaactagggttgttaactgggaagtgatcattatggatgaagcccattttttggatccagctagcatagccgctagaggttgggcagcgcacagagctagggcaaatgaaagtgcaacaatcttgatgacagccacaccgcctgggactagtgatgaatttccacattcaaatggtgaaatagaagatgttcaaacggacatacccagtgagccctggaacacagggcatgactggatcctggctgacaaaaggcccacggcatggttccttccatccatcagagctgcaaatgtcatggctgcctctttgcgtaaggctggaaagagtgtggtggtcctgaacaggaaaacctttgagagagaataccccacgataaagcagaagaaacctgactttatattggccactgacatagctgaaatgggagccaacctttgcgtggagcgagtgctggattgcaggacggcttttaagcctgtgcttgtggatgaagggaggaaggtggcaataaaagggccacttcgtatctccgcatcctctgctgctcaaaggagggggcgcattgggagaaatcccaacagagatggagactcatactactattctgagcctacaagtgaaaataatgcccaccacgtctgctggttggaggcctcaatgctcttggacaacatggaggtgaggggtggaatggtcgccccactctatggcgttgaaggaactaaaacaccagtttcccctggtgaaatgagactgagggatgaccagaggaaagtcttcagagaactagtgaggaattgtgacctgcccgtttggctttcgtggcaagtggccaaggctggtttgaagacgaatgatcgtaagtggtgttttgaaggccctgaggaacatgagatcttgaatgacagcggtgaaacagtgaagtgcagggctcctggaggagcaaagaagcctctgcgcccaaggtggtgtgatgaaagggtgtcatctgaccagagtgcgctgtctgaatttattaagtttgctgaaggtaggaggggagctgctgaagtgctagttgtgctgagtgaactccctgatttcctggctaaaaaaggtggagaggcaatggataccatcagtgtgttcctccactctgaggaaggctctagggcttaccgcaatgcactatcaatgatgcctgaggcaatgacaatagtcatgctgtttatactggctggactactgacatcgggaatggtcatctttttcatgtctcccaaaggcatcagtagaatgtctatggcgatgggcacaatggccggctgtggatatctcatgttccttggaggcgtcaaacccactcacatctcctatgtcatgctcatattctttgtcctgatggtggttgtgatccccgagccagggcaacaaaggtccatccaagacaaccaagtggcatacctcattattggcatcctgacgctggtttcagcggtggcagccaacgagctaggcatgctggagaaaaccaaagaggacctctttgggaagaagaacttaattccatctagtgcttcaccctggagttggccggatcttgacctgaagccaggagctgcctggacagtgtacgttggcattgttacaatgctctctccaatgttgcaccactggatcaaagtcgaatatggcaacctgtctctgtctggaatagcccagtcagcctcagtcctttctttcatggacaaggggataccattcatgaagatgaatatctcggtcataatgctgctggtcagtggctggaattcaataacagtgatgcctctgctctgtggcatagggtgcgccatgctccactggtctctcattttacctggaatcaaagcgcagcagtcaaagcttgcacagagaagggtgttccatggcgttgccaagaaccctgtggttgatgggaatccaacagttgacattgaggaagctcctgaaatgcctgccctttatgagaagaaactggctctatatctccttcttgctctcagcctagcttctgttgccatgtgcagaacgcccttttcattggctgaaggcattgtcctagcatcagctgccttagggccgctcatagagggaaacaccagccttctttggaatggacccatggctgtctccatgacaggagtcatgagggggaatcactatgcttttgtgggagtcatgtacaatctatggaagatgaaaactggacgccgggggagcgcgaatggaaaaactttgggtgaagtctggaagagggaactgaatctgttggacaagcgacagtttgagttgtataaaaggaccgacattgtggaggtggatcgtgatacggcacgcaggcatttggccgaagggaaggtggacaccggggtggcggtctccagggggaccgcaaagttaaggtggttccatgagcgtggctatgtcaagctggaaggtagggtgattgacctggggtgtggccgcggaggctggtgttactacgctgctgcgcaaaaggaagtgagtggggtcaaaggatttactcttggaagagacggccatgagaaacccatgaatgtgcaaagtctgggatggaacatcatcaccttcaaggacaaaactgatatccaccgcctagaaccagtgaaatgtgacacccttttgtgtgacattggagagtcatcatcgtcatcggtcacagagggggaaaggaccgtgagagttcttgatactgtagaaaaatggctggcttgtggggttgacaacttctgtgtgaaggtgttagctccatacatgccagatgttcttgagaaactggaattgctccaaaggaggtttggcggaacagtgatcaggaaccctctctccaggaattccactcatgaaatgtactacgtgtctggagcccgcagcaatgtcacatttactgtgaaccaaacatcccgcctcctgatgaggagaatgaggcgtccaactggaaaagtgaccctggaggctgacgtcatcctcccaattgggacacgcagtgttgagacagacaagggacccctggacaaagaggccatagaagaaagggttgagaggataaaatctgagtacatgacctcttggttttatgacaatgacaacccctacaggacctggcactactgtggctcctatgtcacaaaaacctcaggaagtgcggcgagcatggtaaatggtgttattaaaattctgacatatccatgggacaggatagaggaggtcaccagaatggcaatgactgacacaaccccttttggacagcaaagagtgtttaaagaaaaagttgacaccagagcaaaggatccaccagcgggaactaggaagatcatgaaagttgtcaacaggtggctgttccgccacctggccagagaaaagagccccagactgtgcacaaaggaagaatttattgcaaaagtccgaagtcatgcagccattggagcttacctggaagaacaagaacagtggaagactgccaatgaggctgtccaagacccaaagttctgggaactggtggatgaagaaaggaagctgcaccaacaaggcaggtgtcggacttgtgtgtacaacatgatggggaaaagagagaagaagctgtcagagtttgggaaagcaaagggaagccgtgccatatggtatatgtggctgggagcgcggtatcttgagtttgaggccctgggattcctgaatgaggaccattgggcttccagggaaaactcaggaggaggagtggaaggcattggcttacaatacctaggatatgtgatcagagacctggctgcaatggatggtggtggattctacgcggatgacaccgctggatgggacacgcgcatcacagaggcagaccttgatgatgaacaggagatcttgaactacatgagcccacatcacaaaaaactggcacaagcagtgatggaaatgacatacaagaacaaagtggtgaaagtgttgagaccagccccaggagggaaagcctacatggatgtcataagtcgacgagaccagagaggatccgggcaggtagtgacttatgctctgaacaccatcaccaacttgaaagtccaattgatcagaatggcagaagcagagatggtgatacatcaccaacatgttcaagattgtgatgaatcagttctgaccaggctggaggcatggctcactgagcacggatgtaacagactgaagaggatggcggtgagtggagacgactgtgtggtccggcccatcgatgacaggttcggcctggccctgtcccatctcaacgccatgtccaaggttagaaaggacatatctgaatggcagccatcaaaagggtggaatgattgggagaatgtgcccttctgttcccaccacttccatgaactacagctgaaggatggcaggaggattgtggtgccttgccgagaacaggacgagctcattgggagaggaagggtgtctccaggaaacggctggatgatcaaggaaacagcttgcctcagcaaagcctatgccaacatgtggtcactgatgtattttcacaaaagggacatgaggctactgtcattggctgtttcctcagctgttcccacctcatgggttccacaaggacgcacaacatggtcgattcatgggaaaggggagtggatgaccacggaagacatgcttgaggtgtggaacagagtatggataaccaacaacccacacatgcaggacaagacaatggtgaaaaaatggagagatgtcccttatctaaccaagagacaagacaagctgtgcggatcactgattggaatgaccaatagggccacctgggcctcccacatccatttagtcatccatcgtatccgaacgctgattggacaggagaaatacactgactacctaacagtcatggacaggtattctgtggatgctgacctgcaactgggtgagcttatctgaaacaccatctaacaggaataaccgggatacaaaccacgggtggagaaccggactccccacaacctgaaaccgggatataaaccacggctggagaaccgggctccgcacttaaaatgaaacagaaaccgggataaaaactacggatggagaaccggactccacacattgagacagaagaagttgtcagcccagaaccccacacgagttttgccactgctaagctgtgaggcagtgcaggctgggacagccgacctccaggttgcgaaaaacctggtttctgggacctcccaccccagagtaaaaagaacggagcctccgctaccaccctcccacgtggtggtagaaagacggggtctagaggttagaggagaccctccagggaacaaatagtgggaccatattgacgccagggaaagaccggagtggttctctgcttttcctccagaggtctgtgagcacagtttgctcaagaataagcagacctttggatgacaaacacaaaaccac

SEQ ID NO: 2 - protein, 3724 aa, Yellow fever virus
MSGRKAQGKTLGVNMVRRGVRSLSNKIKQKTKQIGNRPGPSRGVQGFIFFFLFNILTGKKITAHLKRLWKMLDPRQGLAVLRKVKRVVASLMRGLSSRKRRSHDVLTVQFLILGMLLMTGGVTLVRKNRWLLLNVTSEDLGKTFSVGTGNCTTNILEAKYWCPDSMEYNCPNLSPREEPDDIDCWCYGVENVRVAYGKCDSAGRSRRSRRAIDLPTHENHGLKTRQEKWMTGRMGERQLQKIERWFVRNPFFAVTALTIAYLVGSNMTQRVVIALLVLAVGPAYSAHCIGITDRDFIEGVHGGTWVSATLEQDKCVTVMAPDKPSLDISLETVAIDRPAEARKVCYNAVLTHVKINDKCPSTGEAHLAEENEGDNACKRTYSDRGWGNGCGLFGKGSIVACAKFTCAKSMSLFEVDQTKIQYVIRAQLHVGAKQENWNTSIKTLKFDALSGSQEVEFIGYGKATLECQVQTAVDFGNSYIAEMETESWIVDRQWAQDLTLPWQSGSGGVWREMHHLVEFEPPHAATIRVLALGNQEGSLKTALTGAMRVTKDTNDNNLYKLHGGHVSCRVKLSALTLKGTSYKICTDKMFFVKNPTDTGHGTVVMQVKVSKGAPCRIPVIVADDLTAAINKGILVTVNPIASTNDDEVLIEVNPPFGDSYIIVGRGDSRLTYQWHKEGSSIGKLFTQTMKGVERLAVMGDTAWDFSSAGGFFTSVGKGIHTVFGSAFQGLFGGLNWITKVIMGAVLIWVGINTRNMTMSMSMILVGVIMMFLSLGVGADQGCAINFGVSKGEELFTGVVPILVELDGDVNGHKFSVSGEGEGDATYGKLTLKFICTTGKLPVPWPTLVTTLTYGVQCFSRYPDHMKQHDFFKSAMPEGYVQERTIFFKDDGNYKTRAEVKFEGDTLVNRIELKGIDFKEDGNILGHKLEYNYNSHNVYIMADKQKNGIKVNFKIRHNIEDGSVQLADHYQQNTPIGDGPVLLPDNHYLSTQSALSKDPNEKRDHMVLLEFVTAAGITLGMDELYKTSLGKAVHQVFGSVYTTMFGGVSWMIRILIGFLVLWIGTNSRNTSMAMTCIAVGGITLFLGFTVGADQGCAINFGKRELKCGDGIFIFRDSDDWLNKYSYYPEDPVKLASIVKASFEEGKCGLNSVDSLEHEMWRSRADEINAIFEENEVDISVVVQDPKNVYQRGTHPFSRIRDGLQYGWKTWGKNLVFSPGRKNGSFIIDGKSRKECPFSNRVWNSFQIEEFGTGVFTTRVYMDAVFEYTIDCDGSILGAAVNGKKSAHGSPTFWMGSHEVNGTWMIHTLEALDYKECEWPLTHTIGTSVEESEMFMPRSIGGPVSSHNHIPGYKVQTNGPWMQVPLEVKREACPGTSVIIDGNCDGRGKSTRSTTDSGKVIPEWCCRSCTMPPVSFHGSDGCWYPMEIRPRKTHESHLVRSWVTAGEIHAVPFGLVSMMIAMEVVLRKRQGPKQMLVGGVVLLGAMLVGQVTLLDLLKLTVAVGLHFHEMNNGGDAMYMALIAAFSIRPGLLIGFGLRTLWSPRERLVLTLGAAMVEIALGGVMGGLWKYLNAVSLCILTINAVASRKASNTILPLMALLTPVTMAEVRLAAMFFCAMVIIGVLHQNFKDTSMQKTIPLVALTLTSYLGLTQPFLGLCAFLATRIFGRRSIPVNEALAAAGLVGVLAGLAFQEMENFLGPIAVGGLLMMLVSVAGRVDGLELKKLGEVSWEEEAEISGSSARYDVALSEQGEFKLLSEEKVPWDQVVMTSLALVGAALHPFALLLVLAGWLFHVRGARRSGDVLWDIPTPKIIEECEHLEDGIYGIFQSTFLGASQRGVGVAQGGVFHTMWHVTRGAFLVRNGKKLIPSWASVKEDLVAYGGSWKLEGRWDGEEEVQLIAAVPGKNVVNVQTKPSLFKVRNGGEIGAVALDYPSGTSGSPIVNRNGEVIGLYGNGILVGDNSFVSAISQTEVKEEGKEELQEIPTMLKKGMTTVLDFHPGAGKTRRFLPQILAECARRRLRTLVLAPTRVVLSEMKEAFHGLDVKFHTQAFSAHGSGREVIDAMCHATLTYRMLEPTRVVNWEVIIMDEAHFLDPASIAARGWAAHRARANESATILMTATPPGTSDEFPHSNGEIEDVQTDIPSEPWNTGHDWILADKRPTAWFLPSIRAANVMAASLRKAGKSVVVLNRKTFEREYPTIKQKKPDFILATDIAEMGANLCVERVLDCRTAFKPVLVDEGRKVAIKGPLRISASSAAQRRGRIGRNPNRDGDSYYYSEPTSENNAHHVCWLEASMLLDNMEVRGGMVAPLYGVEGTKTPVSPGEMRLRDDQRKVFRELVRNCDLPVWLSWQVAKAGLKTNDRKWCFEGPEEHEILNDSGETVKCRAPGGAKKPLRPRWCDERVSSDQSALSEFIKFAEGRRGAAEVLVVLSELPDFLAKKGGEAMDTISVFLHSEEGSRAYRNALSMMPEAMTIVMLFILAGLLTSGMVIFFMSPKGISRMSMAMGTMAGCGYLMFLGGVKPTHISYVMLIFFVLMVVVIPEPGQQRSIQDNQVAYLIIGILTLVSAVAANELGMLEKTKEDLFGKKNLIPSSASPWSWPDLDLKPGAAWTVYVGIVTMLSPMLHHWIKVEYGNLSLSGIAQSASVLSFMDKGIPFMKMNISVIMLLVSGWNSITVMPLLCGIGCAMLHWSLILPGIKAQQSKLAQRRVFHGVAKNPVVDGNPTVDIEEAPEMPALYEKKLALYLLLALSLASVAMCRTPFSLAEGIVLASAALGPLIEGNTSLLWNGPMAVSMTGVMRGNHYAFVGVMYNLWKMKTGRRGSANGKTLGEVWKRELNLLDKRQFELYKRTDIVEVDRDTARRHLAEGKVDTGVAVSRGTAKLRWFHERGYVKLEGRVIDLGCGRGGWCYYAAAQKEVSGVKGFTLGRDGHEKPMNVQSLGWNIITFKDKTDIHRLEPVKCDTLLCDIGESSSSSVTEGERTVRVLDTVEKWLACGVDNFCVKVLAPYMPDVLEKLELLQRRFGGTVIRNPLSRNSTHEMYYVSGARSNVTFTVNQTSRLLMRRMRRPTGKVTLEADVILPIGTRSVETDKGPLDKEAIEERVERIKSEYMTSWFYDNDNPYRTWHYCGSYVTKTSGSAASMVNGVIKILTYPWDRIEEVTRMAMTDTTPFGQQRVFKEKVDTRAKDPPAGTRKIMKVVNRWLFRHLAREKSPRLCTKEEFIAKVRSHAAIGAYLEEQEQWKTANEAVQDPKFWELVDEERKLHQQGRCRTCVYNMMGKREKKLSEFGKAKGSRAIWYMWLGARYLEFEALGFLNEDHWASRENSGGGVEGIGLQYLGYVIRDLAAMDGGGFYADDTAGWDTRITEADLDDEQEILNYMSPHHKKLAQAVMEMTYKNKVVKVLRPAPGGKAYMDVISRRDQRGSGQVVTYALNTITNLKVQLIRMAEAEMVIHHQHVQDCDESVLTRLEAWLTEHGCNRLKRMAVSGDDCVVRPIDDRFGLALSHLNAMSKVRKDISEWQPSKGWNDWENVPFCSHHFHELQLKDGRRIVVPCREQDELIGRGRVSPGNGWMIKETACLSKAYANMWSLMYFHKRDMRLLSLAVSSAVPTSWVPQGRTTWSIHGKGEWMTTEDMLEVWNRVWITNNPHMQDKTMVKKWRDVPYLTKRQDKLCGSLIGMTNRATWASHIHLVIHRIRTLIGQEKYTDYLTVMDRYSVDADLQLGELI

SEQ ID NO: 3 - DNA, 11890 bp, Yellow fever virus
agtaaatcctgtgtgctaattgaggtgcattggtctgcaaatcgagttgctaggcaataaacacatttggattaattttaatcgttcgttgagcgattagcagagaactgaccagaacatgtctggtcgtaaagctcagggaaaaaccctgggcgtcaatatggtacgacgaggagttcgctccttgtcaaacaaaataaaacaaaaaacaaaacaaattggaaacagacctggaccttcaagaggtgttcaaggatttatctttttctttttgttcaacattttgactggaaaaaagatcacagcccacctaaagaggttgtggaaaatgctggacccaagacaaggcttggctgttctaaggaaagtcaagagagtggtggccagtttgatgagaggattgtcctcaaggaaacgccgttcccatgatgttctgactgtgcaattcctaattttgggaatgctgttgatgaccggtggagtgaccttggtgcggaaaaacagatggttgctcctaaatgtgacatctgaggacctcgggaaaacattctctgtgggcacaggcaactgcacaacaaacattttggaagccaagtactggtgcccagactcaatggaatacaactgtcccaatctcagtccaagagaggagccagatgacattgattgctggtgctatggggtggaaaacgttagagtcgcatatggtaagtgtgactcagcaggcaggtctaggaggtcaagaagggccattgacttgcctacgcatgaaaaccatggtttgaagacccggcaagaaaaatggatgactggaagaatgggtgaaaggcaactccaaaagattgagagatggttcgtgaggaaccccttttttgcagtgacggctctgaccattgcctaccttgtgggaagcaacatgacgcaacgagtcgtgattgccctactggtcttggctgttggtccggcctactcagctcactgcattggaattactgacagggatttcattgagggggtgcatggaggaacttgggtttcagctaccctggagcaagacaagtgtgtcactgttatggcccctgacaagccttcattggacatctcactagagacagtagccattgatagacctgctgaggcgaggaaagtgtgttacaatgcagttctcactcatgtgaagattaatgacaagtgccccagcactggagaggcccacctagctgaagagaacgaaggggacaatgcgtgcaagcgcacttattctgatagaggctggggcaatggctgtggcctatttgggaaagggagcattgtggcatgcgccaaattcacttgtgccaaatccatgagtttgtttgaggttgatcagaccaaaattcagtatgtcatcagagcacaattgcatgtaggggccaagcaggaaaattggaataccagcattaagactctcaagtttgatgccctgtcaggctcccaggaagtcgagttcattgggtatggaaaagctacactggaatgccaggtgcaaactgcggtggactttggtaacagttacatcgctgagatggaaacagagagctggatagtggacagacagtgggcccaggacttgaccctgccatggcagagtggaagtggcggggtgtggagagagatgcatcatcttgtcgaatttgaacctccgcatgccgccactatcagagtactggccctgggaaaccaggaaggctccttgaaaacagctcttactggcgcaatgagggttacaaaggacacaaatgacaacaacctttacaaactacatggtggacatgtttcttgcagagtgaaattgtcagctttgacactcaaggggacatcctacaaaatatgcactgacaaaatgttttttgtcaagaacccaactgacactggccatggcactgttgtgatgcaggtgaaagtgtcaaaaggagccccctgcaggattccagtgatagtagctgatgatcttacagcggcaatcaataaaggcattttggttacagttaaccccatcgcctcaaccaatgatgatgaagtgctgattgaggtgaacccaccttttggagacagctacattatcgttgggagaggagattcacgtctcacttaccagtggcacaaagagggaagctcaataggaaagttgttcactcagaccatgaaaggcgtggaacgcctggccgtcatgggagacaccgcctgggatttcagctccgctggagggttcttcacttcggttgggaaaggaattcatacggtgtttggctctgcctttcaggggctatttggcggcttgaactggataacaaaggtcatcatgggggcggtacttatatgggttggcatcaacacaagaaacatgacaatgtccatgagcatgatcttggtaggagtgatcatgatgtttttgtctctaggagttggggcggatcaaggatgcgccatcaactttggcgtgagcaagggcgaggagctgttcaccggggtggtgcccatcctggtcgagctggacggcgacgtaaacggccacaagttcagcgtgtccggcgagggcgagggcgatgccacctacggcaagctgaccctgaagttcatctgcaccaccggcaagctgcccgtgccctggcccaccctcgtgaccaccctgacctacggcgtgcagtgcttcagccgctaccccgaccacatgaagcagcacgacttcttcaagtccgccatgcccgaaggctacgtccaggagcgcaccatcttcttcaaggacgacggcaactacaagacccgcgccgaggtgaagttcgagggcgacaccctggtgaaccgcatcgagctgaagggcatcgacttcaaggaggacggcaacatcctggggcacaagctggagtacaactacaacagccacaacgtctatatcatggccgacaagcagaagaacggcatcaaggtgaacttcaagatccgccacaacatcgaggacggcagcgtgcagctcgccgaccactaccagcagaacacccccatcggcgacggccccgtgctgctgcccgacaaccactacctgagcacccagtccgccctgagcaaagaccccaacgagaagcgcgatcacatggtcctgctggagttcgtgaccgccgccgggatcactctcggcatggacgagctgtacaagaagatgtttgagtccacatacagaggtgcaaaacgaatggccattctaggtgaaacagcttgggattttggttccgttggtggactgttcacatcattgggaaaggctgtgcaccaggtttttggaagtgtgtatacaaccatgtttggaggagtctcatggatgattagaatcctaattgggttcttagtgttgtggattggcacgaactccaggaacacttcaatggctatgacgtgcatagctgttggaggaatcactctgtttctgggcttcacagttggcgccgatcaaggatgcgccatcaactttggcaagagagagctcaagtgcggagatggtatcttcatatttagagactctgatgactggctgaacaagtactcatactatccagaagatcctgtgaagcttgcatcaatagtgaaagcctcttttgaagaagggaagtgtggcctaaattcagttgactcccttgagcatgagatgtggagaagcagggcagatgagatcaatgccatttttgaggaaaacgaggtggacatttctgttgtcgtgcaggatccaaagaatgtttaccagagaggaactcatccattttccagaattcgggatggtctgcagtatggttggaagacttggggtaagaaccttgtgttctccccagggaggaagaatggaagcttcatcatagatggaaagtccaggaaagaatgcccgttttcaaaccgggtctggaattctttccagatagaggagtttgggacgggagtgttcaccacacgcgtgtacatggacgcagtctttgaatacaccatagactgcgatggatctatcttgggtgcagcggtgaacggaaaaaagagtgcccatggctctccaacattttggatgggaagtcatgaagtaaatgggacatggatgatccacaccttggaggcattagattacaaggagtgtgagtggccactgacacatacgattggaacatcagttgaagagagtgaaatgttcatgccgagatcaatcggaggcccagttagctctcacaatcatatccctggatacaaggttcagacgaacggaccttggatgcaggtaccactagaagtgaagagagaagcttgcccagggactagcgtgatcattgatggcaactgtgatggacggggaaaatcaaccagatccaccacggatagcgggaaagttattcctgaatggtgttgccgctcctgcacaatgccgcctgtgagcttccatggtagtgatgggtgttggtatcccatggaaattaggccaaggaaaacgcatgaaagccatctggtgcgctcctgggttacagctggagaaatacatgctgtcccttttggtttggtgagcatgatgatagcaatggaagtggtcctaaggaaaagacagggaccaaagcaaatgttggttggaggagtagtgctcttgggagcaatgctggtcgggcaagtaactctccttgatttgctgaaactcacagtggctgtgggattgcatttccatgagatgaacaatggaggagacgccatgtatatggcgttgattgctgccttttcaatcagaccagggctgctcatcggctttgggctcaggaccctatggagccctcgggaacgccttgtgctgaccctaggagcagccatggtggagattgccttgggtggcgtgatgggcggcctgtggaagtatctaaatgcagtttctctctgcatcctgacaataaatgctgttgcttctaggaaagcatcaaataccatcttgcccctcatggctctgttgacacctgtcactatggctgaggtgagacttgccgcaatgttcttttgtgccatggttatcataggggtccttcaccagaatttcaaggacacctccatgcagaagactatacctctggtggccctcacactcacatcttacctgggcttgacacaaccttttttgggcctgtgtgcatttctggcaacccgcatatttgggcgaaggagtatcccagtgaatgaggcactcgcagcagctggtctagtgggagtgctggcaggactggcttttcaggagatggagaacttccttggtccgattgcagttggaggactcctgatgatgctggttagcgtggctgggagggtggatgggctagagctcaagaagcttggtgaagtttcatgggaagaggaggcggagatcagcgggagttccgcccgctatgatgtggcactcagtgaacaaggggagttcaagctgctttctgaagagaaagtgccatgggaccaggttgtgatgacctcgctggccttggttggggctgccctccatccatttgctcttctgctggtccttgctgggtggctgtttcatgtcaggggagctaggagaagtggggatgtcttgtgggatattcccactcctaagatcatcgaggaatgtgaacatctggaggatgggatttatggcatattccagtcaaccttcttgggggcctcccagcgaggagtgggagtggcacagggaggggtgttccacacaatgtggcatgtcacaagaggagctttccttgtcaggaatggcaagaagttgattccatcttgggcttcagtaaaggaagaccttgtcgcctatggtggctcatggaagttggaaggcagatgggatggagaggaagaggtccagttgatcgcggctgttccaggaaagaacgtggtcaacgtccagacaaaaccgagcttgttcaaagtgaggaatgggggagaaatcggggctgtcgctcttgactatccgagtggcacttcaggatctcctattgttaacaggaacggagaggtgattgggctgtacggcaatggcatccttgtcggtgacaactccttcgtgtccgccatatcccagactgaggtgaaggaagaaggaaaggaggagctccaagagatcccgacaatgctaaagaaaggaatgacaactgtccttgattttcatcctggagctgggaagacaagacgtttcctcccacagatcttggccgagtgcgcacggagacgcttgcgcactcttgtgttggcccccaccagggttgttctttctgaaatgaaggaggcttttcacggcctggacgtgaaattccacacacaggctttttccgctcacggcagcgggagagaagtcattgatgccatgtgccatgccaccctaacttacaggatgttggaaccaactagggttgttaactgggaagtgatcattatggatgaagcccattttttggatccagctagcatagccgctagaggttgggcagcgcacagagctagggcaaatgaaagtgcaacaatcttgatgacagccacaccgcctgggactagtgatgaatttccacattcaaatggtgaaatagaagatgttcaaacggacatacccagtgagccctggaacacagggcatgactggatcctggctgacaaaaggcccacggcatggttccttccatccatcagagctgcaaatgtcatggctgcctctttgcgtaaggctggaaagagtgtggtggtcctgaacaggaaaacctttgagagagaataccccacgataaagcagaagaaacctgactttatattggccactgacatagctgaaatgggagccaacctttgcgtggagcgagtgctggattgcaggacggcttttaagcctgtgcttgtggatgaagggaggaaggtggcaataaaagggccacttcgtatctccgcatcctctgctgctcaaaggagggggcgcattgggagaaatcccaacagagatggagactcatactactattctgagcctacaagtgaaaataatgcccaccacgtctgctggttggaggcctcaatgctcttggacaacatggaggtgaggggtggaatggtcgccccactctatggcgttgaaggaactaaaacaccagtttcccctggtgaaatgagactgagggatgaccagaggaaagtcttcagagaactagtgaggaattgtgacctgcccgtttggctttcgtggcaagtggccaaggctggtttgaagacgaatgatcgtaagtggtgttttgaaggccctgaggaacatgagatcttgaatgacagcggtgaaacagtgaagtgcagggctcctggaggagcaaagaagcctctgcgcccaaggtggtgtgatgaaagggtgtcatctgaccagagtgcgctgtctgaatttattaagtttgctgaaggtaggaggggagctgctgaagtgctagttgtgctgagtgaactccctgatttcctggctaaaaaaggtggagaggcaatggataccatcagtgtgttcctccactctgaggaaggctctagggcttaccgcaatgcactatcaatgatgcctgaggcaatgacaatagtcatgctgtttatactggctggactactgacatcgggaatggtcatctttttcatgtctcccaaaggcatcagtagaatgtctatggcgatgggcacaatggccggctgtggatatctcatgttccttggaggcgtcaaacccactcacatctcctatgtcatgctcatattctttgtcctgatggtggttgtgatccccgagccagggcaacaaaggtccatccaagacaaccaagtggcatacctcattattggcatcctgacgctggtttcagcggtggcagccaacgagctaggcatgctggagaaaaccaaagaggacctctttgggaagaagaacttaattccatctagtgcttcaccctggagttggccggatcttgacctgaagccaggagctgcctggacagtgtacgttggcattgttacaatgctctctccaatgttgcaccactggatcaaagtcgaatatggcaacctgtctctgtctggaatagcccagtcagcctcagtcctttctttcatggacaaggggataccattcatgaagatgaatatctcggtcataatgctgctggtcagtggctggaattcaataacagtgatgcctctgctctgtggcatagggtgcgccatgctccactggtctctcattttacctggaatcaaagcgcagcagtcaaagcttgcacagagaagggtgttccatggcgttgccaagaaccctgtggttgatgggaatccaacagttgacattgaggaagctcctgaaatgcctgccctttatgagaagaaactggctctatatctccttcttgctctcagcctagcttctgttgccatgtgcagaacgcccttttcattggctgaaggcattgtcctagcatcagctgccttagggccgctcatagagggaaacaccagccttctttggaatggacccatggctgtctccatgacaggagtcatgagggggaatcactatgcttttgtgggagtcatgtacaatctatggaagatgaaaactggacgccgggggagcgcgaatggaaaaactttgggtgaagtctggaagagggaactgaatctgttggacaagcgacagtttgagttgtataaaaggaccgacattgtggaggtggatcgtgatacggcacgcaggcatttggccgaagggaaggtggacaccggggtggcggtctccagggggaccgcaaagttaaggtggttccatgagcgtggctatgtcaagctggaaggtagggtgattgacctggggtgtggccgcggaggctggtgttactacgctgctgcgcaaaaggaagtgagtggggtcaaaggatttactcttggaagagacggccatgagaaacccatgaatgtgcaaagtctgggatggaacatcatcaccttcaaggacaaaactgatatccaccgcctagaaccagtgaaatgtgacacccttttgtgtgacattggagagtcatcatcgtcatcggtcacagagggggaaaggaccgtgagagttcttgatactgtagaaaaatggctggcttgtggggttgacaacttctgtgtgaaggtgttagctccatacatgccagatgttcttgagaaactggaattgctccaaaggaggtttggcggaacagtgatcaggaaccctctctccaggaattccactcatgaaatgtactacgtgtctggagcccgcagcaatgtcacatttactgtgaaccaaacatcccgcctcctgatgaggagaatgaggcgtccaactggaaaagtgaccctggaggctgacgtcatcctcccaattgggacacgcagtgttgagacagacaagggacccctggacaaagaggccatagaagaaagggttgagaggataaaatctgagtacatgacctcttggttttatgacaatgacaacccctacaggacctggcactactgtggctcctatgtcacaaaaacctcaggaagtgcggcgagcatggtaaatggtgttattaaaattctgacatatccatgggacaggatagaggaggtcaccagaatggcaatgactgacacaaccccttttggacagcaaagagtgtttaaagaaaaagttgacaccagagcaaaggatccaccagcgggaactaggaagatcatgaaagttgtcaacaggtggctgttccgccacctggccagagaaaagagccccagactgtgcacaaaggaagaatttattgcaaaagtccgaagtcatgcagccattggagcttacctggaagaacaagaacagtggaagactgccaatgaggctgtccaagacccaaagttctgggaactggtggatgaagaaaggaagctgcaccaacaaggcaggtgtcggacttgtgtgtacaacatgatggggaaaagagagaagaagctgtcagagtttgggaaagcaaagggaagccgtgccatatggtatatgtggctgggagcgcggtatcttgagtttgaggccctgggattcctgaatgaggaccattgggcttccagggaaaactcaggaggaggagtggaaggcattggcttacaatacctaggatatgtgatcagagacctggctgcaatggatggtggtggattctacgcggatgacaccgctggatgggacacgcgcatcacagaggcagaccttgatgatgaacaggagatcttgaactacatgagcccacatcacaaaaaactggcacaagcagtgatggaaatgacatacaagaacaaagtggtgaaagtgttgagaccagccccaggagggaaagcctacatggatgtcataagtcgacgagaccagagaggatccgggcaggtagtgacttatgctctgaacaccatcaccaacttgaaagtccaattgatcagaatggcagaagcagagatggtgatacatcaccaacatgttcaagattgtgatgaatcagttctgaccaggctggaggcatggctcactgagcacggatgtaacagactgaagaggatggcggtgagtggagacgactgtgtggtccggcccatcgatgacaggttcggcctggccctgtcccatctcaacgccatgtccaaggttagaaaggacatatctgaatggcagccatcaaaagggtggaatgattgggagaatgtgcccttctgttcccaccacttccatgaactacagctgaaggatggcaggaggattgtggtgccttgccgagaacaggacgagctcattgggagaggaagggtgtctccaggaaacggctggatgatcaaggaaacagcttgcctcagcaaagcctatgccaacatgtggtcactgatgtattttcacaaaagggacatgaggctactgtcattggctgtttcctcagctgttcccacctcatgggttccacaaggacgcacaacatggtcgattcatgggaaaggggagtggatgaccacggaagacatgcttgaggtgtggaacagagtatggataaccaacaacccacacatgcaggacaagacaatggtgaaaaaatggagagatgtcccttatctaaccaagagacaagacaagctgtgcggatcactgattggaatgaccaatagggccacctgggcctcccacatccatttagtcatccatcgtatccgaacgctgattggacaggagaaatacactgactacctaacagtcatggacaggtattctgtggatgctgacctgcaactgggtgagcttatctgaaacaccatctaacaggaataaccgggatacaaaccacgggtggagaaccggactccccacaacctgaaaccgggatataaaccacggctggagaaccgggctccgcacttaaaatgaaacagaaaccgggataaaaactacggatggagaaccggactccacacattgagacagaagaagttgtcagcccagaaccccacacgagttttgccactgctaagctgtgaggcagtgcaggctgggacagccgacctccaggttgcgaaaaacctggtttctgggacctcccaccccagagtaaaaagaacggagcctccgctaccaccctcccacgtggtggtagaaagacggggtctagaggttagaggagaccctccagggaacaaatagtgggaccatattgacgccagggaaagaccggagtggttctctgcttttcctccagaggtctgtgagcacagtttgctcaagaataagcagacctttggatgacaaacacaaaaccac

SEQ ID NO: 4 - protein, 3754 aa, Yellow fever virus
MSGRKAQGKTLGVNMVRRGVRSLSNKIKQKTKQIGNRPGPSRGVQGFIFFFLFNILTGKKITAHLKRLWKMLDPRQGLAVLRKVKRVVASLMRGLSSRKRRSHDVLTVQFLILGMLLMTGGVTLVRKNRWLLLNVTSEDLGKTFSVGTGNCTTNILEAKYWCPDSMEYNCPNLSPREEPDDIDCWCYGVENVRVAYGKCDSAGRSRRSRRAIDLPTHENHGLKTRQEKWMTGRMGERQLQKIERWFVRNPFFAVTALTIAYLVGSNMTQRVVIALLVLAVGPAYSAHCIGITDRDFIEGVHGGTWVSATLEQDKCVTVMAPDKPSLDISLETVAIDRPAEARKVCYNAVLTHVKINDKCPSTGEAHLAEENEGDNACKRTYSDRGWGNGCGLFGKGSIVACAKFTCAKSMSLFEVDQTKIQYVIRAQLHVGAKQENWNTSIKTLKFDALSGSQEVEFIGYGKATLECQVQTAVDFGNSYIAEMETESWIVDRQWAQDLTLPWQSGSGGVWREMHHLVEFEPPHAATIRVLALGNQEGSLKTALTGAMRVTKDTNDNNLYKLHGGHVSCRVKLSALTLKGTSYKICTDKMFFVKNPTDTGHGTVVMQVKVSKGAPCRIPVIVADDLTAAINKGILVTVNPIASTNDDEVLIEVNPPFGDSYIIVGRGDSRLTYQWHKEGSSIGKLFTQTMKGVERLAVMGDTAWDFSSAGGFFTSVGKGIHTVFGSAFQGLFGGLNWITKVIMGAVLIWVGINTRNMTMSMSMILVGVIMMFLSLGVGADQGCAINFGVSKGEELFTGVVPILVELDGDVNGHKFSVSGEGEGDATYGKLTLKFICTTGKLPVPWPTLVTTLTYGVQCFSRYPDHMKQHDFFKSAMPEGYVQERTIFFKDDGNYKTRAEVKFEGDTLVNRIELKGIDFKEDGNILGHKLEYNYNSHNVYIMADKQKNGIKVNFKIRHNIEDGSVQLADHYQQNTPIGDGPVLLPDNHYLSTQSALSKDPNEKRDHMVLLEFVTAAGITLGMDELYKKMFESTYRGAKRMAILGETAWDFGSVGGLFTSLGKAVHQVFGSVYTTMFGGVSWMIRILIGFLVLWIGTNSRNTSMAMTCIAVGGITLFLGFTVGADQGCAINFGKRELKCGDGIFIFRDSDDWLNKYSYYPEDPVKLASIVKASFEEGKCGLNSVDSLEHEMWRSRADEINAIFEENEVDISVVVQDPKNVYQRGTHPFSRIRDGLQYGWKTWGKNLVFSPGRKNGSFIIDGKSRKECPFSNRVWNSFQIEEFGTGVFTTRVYMDAVFEYTIDCDGSILGAAVNGKKSAHGSPTFWMGSHEVNGTWMIHTLEALDYKECEWPLTHTIGTSVEESEMFMPRSIGGPVSSHNHIPGYKVQTNGPWMQVPLEVKREACPGTSVIIDGNCDGRGKSTRSTTDSGKVIPEWCCRSCTMPPVSFHGSDGCWYPMEIRPRKTHESHLVRSWVTAGEIHAVPFGLVSMMIAMEVVLRKRQGPKQMLVGGVVLLGAMLVGQVTLLDLLKLTVAVGLHFHEMNNGGDAMYMALIAAFSIRPGLLIGFGLRTLWSPRERLVLTLGAAMVEIALGGVMGGLWKYLNAVSLCILTINAVASRKASNTILPLMALLTPVTMAEVRLAAMFFCAMVIIGVLHQNFKDTSMQKTIPLVALTLTSYLGLTQPFLGLCAFLATRIFGRRSIPVNEALAAAGLVGVLAGLAFQEMENFLGPIAVGGLLMMLVSVAGRVDGLELKKLGEVSWEEEAEISGSSARYDVALSEQGEFKLLSEEKVPWDQVVMTSLALVGAALHPFALLLVLAGWLFHVRGARRSGDVLWDIPTPKIIEECEHLEDGIYGIFQSTFLGASQRGVGVAQGGVFHTMWHVTRGAFLVRNGKKLIPSWASVKEDLVAYGGSWKLEGRWDGEEEVQLIAAVPGKNVVNVQTKPSLFKVRNGGEIGAVALDYPSGTSGSPIVNRNGEVIGLYGNGILVGDNSFVSAISQTEVKEEGKEELQEIPTMLKKGMTTVLDFHPGAGKTRRFLPQILAECARRRLRTLVLAPTRVVLSEMKEAFHGLDVKFHTQAFSAHGSGREVIDAMCHATLTYRMLEPTRVVNWEVIIMDEAHFLDPASIAARGWAAHRARANESATILMTATPPGTSDEFPHSNGEIEDVQTDIPSEPWNTGHDWILADKRPTAWFLPSIRAANVMAASLRKAGKSVVVLNRKTFEREYPTIKQKKPDFILATDIAEMGANLCVERVLDCRTAFKPVLVDEGRKVAIKGPLRISASSAAQRRGRIGRNPNRDGDSYYYSEPTSENNAHHVCWLEASMLLDNMEVRGGMVAPLYGVEGTKTPVSPGEMRLRDDQRKVFRELVRNCDLPVWLSWQVAKAGLKTNDRKWCFEGPEEHEILNDSGETVKCRAPGGAKKPLRPRWCDERVSSDQSALSEFIKFAEGRRGAAEVLVVLSELPDFLAKKGGEAMDTISVFLHSEEGSRAYRNALSMMPEAMTIVMLFILAGLLTSGMVIFFMSPKGISRMSMAMGTMAGCGYLMFLGGVKPTHISYVMLIFFVLMVVVIPEPGQQRSIQDNQVAYLIIGILTLVSAVAANELGMLEKTKEDLFGKKNLIPSSASPWSWPDLDLKPGAAWTVYVGIVTMLSPMLHHWIKVEYGNLSLSGIAQSASVLSFMDKGIPFMKMNISVIMLLVSGWNSITVMPLLCGIGCAMLHWSLILPGIKAQQSKLAQRRVFHGVAKNPVVDGNPTVDIEEAPEMPALYEKKLALYLLLALSLASVAMCRTPFSLAEGIVLASAALGPLIEGNTSLLWNGPMAVSMTGVMRGNHYAFVGVMYNLWKMKTGRRGSANGKTLGEVWKRELNLLDKRQFELYKRTDIVEVDRDTARRHLAEGKVDTGVAVSRGTAKLRWFHERGYVKLEGRVIDLGCGRGGWCYYAAAQKEVSGVKGFTLGRDGHEKPMNVQSLGWNIITFKDKTDIHRLEPVKCDTLLCDIGESSSSSVTEGERTVRVLDTVEKWLACGVDNFCVKVLAPYMPDVLEKLELLQRRFGGTVIRNPLSRNSTHEMYYVSGARSNVTFTVNQTSRLLMRRMRRPTGKVTLEADVILPIGTRSVETDKGPLDKEAIEERVERIKSEYMTSWFYDNDNPYRTWHYCGSYVTKTSGSAASMVNGVIKILTYPWDRIEEVTRMAMTDTTPFGQQRVFKEKVDTRAKDPPAGTRKIMKVVNRWLFRHLAREKSPRLCTKEEFIAKVRSHAAIGAYLEEQEQWKTANEAVQDPKFWELVDEERKLHQQGRCRTCVYNMMGKREKKLSEFGKAKGSRAIWYMWLGARYLEFEALGFLNEDHWASRENSGGGVEGIGLQYLGYVIRDLAAMDGGGFYADDTAGWDTRITEADLDDEQEILNYMSPHHKKLAQAVMEMTYKNKVVKVLRPAPGGKAYMDVISRRDQRGSGQVVTYALNTITNLKVQLIRMAEAEMVIHHQHVQDCDESVLTRLEAWLTEHGCNRLKRMAVSGDDCVVRPIDDRFGLALSHLNAMSKVRKDISEWQPSKGWNDWENVPFCSHHFHELQLKDGRRIVVPCREQDELIGRGRVSPGNGWMIKETACLSKAYANMWSLMYFHKRDMRLLSLAVSSAVPTSWVPQGRTTWSIHGKGEWMTTEDMLEVWNRVWITNNPHMQDKTMVKKWRDVPYLTKRQDKLCGSLIGMTNRATWASHIHLVIHRIRTLIGQEKYTDYLTVMDRYSVDADLQLGELI

SEQ ID NO: 5 - DNA, 11941 bp, Yellow fever virus
agtaaatcctgtgtgctaattgaggtgcattggtctgcaaatcgagttgctaggcaataaacacatttggattaattttaatcgttcgttgagcgattagcagagaactgaccagaacatgtctggtcgtaaagctcagggaaaaaccctgggcgtcaatatggtacgacgaggagttcgctccttgtcaaacaaaataaaacaaaaaacaaaacaaattggaaacagacctggaccttcaagaggtgttcaaggatttatctttttctttttgttcaacattttgactggaaaaaagatcacagcccacctaaagaggttgtggaaaatgctggacccaagacaaggcttggctgttctaaggaaagtcaagagagtggtggccagtttgatgagaggattgtcctcaaggaaacgccgttcccatgatgttctgactgtgcaattcctaattttgggaatgctgttgatgaccggtggagtgaccttggtgcggaaaaacagatggttgctcctaaatgtgacatctgaggacctcgggaaaacattctctgtgggcacaggcaactgcacaacaaacattttggaagccaagtactggtgcccagactcaatggaatacaactgtcccaatctcagtccaagagaggagccagatgacattgattgctggtgctatggggtggaaaacgttagagtcgcatatggtaagtgtgactcagcaggcaggtctaggaggtcaagaagggccattgacttgcctacgcatgaaaaccatggtttgaagacccggcaagaaaaatggatgactggaagaatgggtgaaaggcaactccaaaagattgagagatggttcgtgaggaaccccttttttgcagtgacggctctgaccattgcctaccttgtgggaagcaacatgacgcaacgagtcgtgattgccctactggtcttggctgttggtccggcctactcagctcactgcattggaattactgacagggatttcattgagggggtgcatggaggaacttgggtttcagctaccctggagcaagacaagtgtgtcactgttatggcccctgacaagccttcattggacatctcactagagacagtagccattgatagacctgctgaggcgaggaaagtgtgttacaatgcagttctcactcatgtgaagattaatgacaagtgccccagcactggagaggcccacctagctgaagagaacgaaggggacaatgcgtgcaagcgcacttattctgatagaggctggggcaatggctgtggcctatttgggaaagggagcattgtggcatgcgccaaattcacttgtgccaaatccatgagtttgtttgaggttgatcagaccaaaattcagtatgtcatcagagcacaattgcatgtaggggccaagcaggaaaattggaataccagcattaagactctcaagtttgatgccctgtcaggctcccaggaagtcgagttcattgggtatggaaaagctacactggaatgccaggtgcaaactgcggtggactttggtaacagttacatcgctgagatggaaacagagagctggatagtggacagacagtgggcccaggacttgaccctgccatggcagagtggaagtggcggggtgtggagagagatgcatcatcttgtcgaatttgaacctccgcatgccgccactatcagagtactggccctgggaaaccaggaaggctccttgaaaacagctcttactggcgcaatgagggttacaaaggacacaaatgacaacaacctttacaaactacatggtggacatgtttcttgcagagtgaaattgtcagctttgacactcaaggggacatcctacaaaatatgcactgacaaaatgttttttgtcaagaacccaactgacactggccatggcactgttgtgatgcaggtgaaagtgtcaaaaggagccccctgcaggattccagtgatagtagctgatgatcttacagcggcaatcaataaaggcattttggttacagttaaccccatcgcctcaaccaatgatgatgaagtgctgattgaggtgaacccaccttttggagacagctacattatcgttgggagaggagattcacgtctcacttaccagtggcacaaagagggaagctcaataggaaagttgttcactcagaccatgaaaggcgtggaacgcctggccgtcatgggagacaccgcctgggatttcagctccgctggagggttcttcacttcggttgggaaaggaattcatacggtgtttggctctgcctttcaggggctatttggcggcttgaactggataacaaaggtcatcatgggggcggtacttatatgggttggcatcaacacaagaaacatgacaatgtccatgagcatgatcttggtaggagtgatcatgatgtttttgtctctaggagttggggcggatcaaggatgcgccatcaacttcggccgaaagggatcacaaacctccaacacaactaaatgggctcctcccggacaaggaagtccaggtagcaagggcgaggagctgttcaccggggtggtgcccatcctggtcgagctggacggcgacgtaaacggccacaagttcagcgtgtccggcgagggcgagggcgatgccacctacggcaagctgaccctgaagttcatctgcaccaccggcaagctgcccgtgccctggcccaccctcgtgaccaccctgacctacggcgtgcagtgcttcagccgctaccccgaccacatgaagcagcacgacttcttcaagtccgccatgcccgaaggctacgtccaggagcgcaccatcttcttcaaggacgacggcaactacaagacccgcgccgaggtgaagttcgagggcgacaccctggtgaaccgcatcgagctgaagggcatcgacttcaaggaggacggcaacatcctggggcacaagctggagtacaactacaacagccacaacgtctatatcatggccgacaagcagaagaacggcatcaaggtgaacttcaagatccgccacaacatcgaggacggcagcgtgcagctcgccgaccactaccagcagaacacccccatcggcgacggccccgtgctgctgcccgacaaccactacctgagcacccagtccgccctgagcaaagaccccaacgagaagcgcgatcacatggtcctgctggagttcgtgaccgccgccgggatcactctcggcatggacgagctgtacaagggtagcagtccactgtctcatcgcagtaaaaggagcctatcctgtcggccacccatggtcaaagagggaagctcaataggaacatcattgggaaaggctgtgcaccaggtttttggaagtgtgtatacaaccatgtttggaggagtctcatggatgattagaatcctaattgggttcttagtgttgtggattggcacgaactcaaggaacacttcaatggctatgacgtgcatagctgttggaggaatcactctgtttctgggcttcacagttggcgccgatcaaggatgcgccatcaactttggcaagagagagctcaagtgcggagatggtatcttcatatttagagactctgatgactggctgaacaagtactcatactatccagaagatcctgtgaagcttgcatcaatagtgaaagcctcttttgaagaagggaagtgtggcctaaattcagttgactcccttgagcatgagatgtggagaagcagggcagatgagatcaatgccatttttgaggaaaacgaggtggacatttctgttgtcgtgcaggatccaaagaatgtttaccagagaggaactcatccattttccagaattcgggatggtctgcagtatggttggaagacttggggtaagaaccttgtgttctccccagggaggaagaatggaagcttcatcatagatggaaagtccaggaaagaatgcccgttttcaaaccgggtctggaattctttccagatagaggagtttgggacgggagtgttcaccacacgcgtgtacatggacgcagtctttgaatacaccatagactgcgatggatctatcttgggtgcagcggtgaacggaaaaaagagtgcccatggctctccaacattttggatgggaagtcatgaagtaaatgggacatggatgatccacaccttggaggcattagattacaaggagtgtgagtggccactgacacatacgattggaacatcagttgaagagagtgaaatgttcatgccgagatcaatcggaggcccagttagctctcacaatcatatccctggatacaaggttcagacgaacggaccttggatgcaggtaccactagaagtgaagagagaagcttgcccagggactagcgtgatcattgatggcaactgtgatggacggggaaaatcaaccagatccaccacggatagcgggaaagttattcctgaatggtgttgccgctcctgcacaatgccgcctgtgagcttccatggtagtgatgggtgttggtatcccatggaaattaggccaaggaaaacgcatgaaagccatctggtgcgctcctgggttacagctggagaaatacatgctgtcccttttggtttggtgagcatgatgatagcaatggaagtggtcctaaggaaaagacagggaccaaagcaaatgttggttggaggagtagtgctcttgggagcaatgctggtcgggcaagtaactctccttgatttgctgaaactcacagtggctgtgggattgcatttccatgagatgaacaatggaggagacgccatgtatatggcgttgattgctgccttttcaatcagaccagggctgctcatcggctttgggctcaggaccctatggagccctcgggaacgccttgtgctgaccctaggagcagccatggtggagattgccttgggtggcgtgatgggcggcctgtggaagtatctaaatgcagtttctctctgcatcctgacaataaatgctgttgcttctaggaaagcatcaaataccatcttgcccctcatggctctgttgacacctgtcactatggctgaggtgagacttgccgcaatgttcttttgtgccatggttatcataggggtccttcaccagaatttcaaggacacctccatgcagaagactatacctctggtggccctcacactcacatcttacctgggcttgacacaaccttttttgggcctgtgtgcatttctggcaacccgcatatttgggcgaaggagtatcccagtgaatgaggcactcgcagcagctggtctagtgggagtgctggcaggactggcttttcaggagatggagaacttccttggtccgattgcagttggaggactcctgatgatgctggttagcgtggctgggagggtggatgggctagagctcaagaagcttggtgaagtttcatgggaagaggaggcggagatcagcgggagttccgcccgctatgatgtggcactcagtgaacaaggggagttcaagctgctttctgaagagaaagtgccatgggaccaggttgtgatgacctcgctggccttggttggggctgccctccatccatttgctcttctgctggtccttgctgggtggctgtttcatgtcaggggagctaggagaagtggggatgtcttgtgggatattcccactcctaagatcatcgaggaatgtgaacatctggaggatgggatttatggcatattccagtcaaccttcttgggggcctcccagcgaggagtgggagtggcacagggaggggtgttccacacaatgtggcatgtcacaagaggagctttccttgtcaggaatggcaagaagttgattccatcttgggcttcagtaaaggaagaccttgtcgcctatggtggctcatggaagttggaaggcagatgggatggagaggaagaggtccagttgatcgcggctgttccaggaaagaacgtggtcaacgtccagacaaaaccgagcttgttcaaagtgaggaatgggggagaaatcggggctgtcgctcttgactatccgagtggcacttcaggatctcctattgttaacaggaacggagaggtgattgggctgtacggcaatggcatccttgtcggtgacaactccttcgtgtccgccatatcccagactgaggtgaaggaagaaggaaaggaggagctccaagagatcccgacaatgctaaagaaaggaatgacaactgtccttgattttcatcctggagctgggaagacaagacgtttcctcccacagatcttggccgagtgcgcacggagacgcttgcgcactcttgtgttggcccccaccagggttgttctttctgaaatgaaggaggcttttcacggcctggacgtgaaattccacacacaggctttttccgctcacggcagcgggagagaagtcattgatgccatgtgccatgccaccctaacttacaggatgttggaaccaactagggttgttaactgggaagtgatcattatggatgaagcccattttttggatccagctagcatagccgctagaggttgggcagcgcacagagctagggcaaatgaaagtgcaacaatcttgatgacagccacaccgcctgggactagtgatgaatttccacattcaaatggtgaaatagaagatgttcaaacggacatacccagtgagccctggaacacagggcatgactggatcctggctgacaaaaggcccacggcatggttccttccatccatcagagctgcaaatgtcatggctgcctctttgcgtaaggctggaaagagtgtggtggtcctgaacaggaaaacctttgagagagaataccccacgataaagcagaagaaacctgactttatattggccactgacatagctgaaatgggagccaacctttgcgtggagcgagtgctggattgcaggacggcttttaagcctgtgcttgtggatgaagggaggaaggtggcaataaaagggccacttcgtatctccgcatcctctgctgctcaaaggagggggcgcattgggagaaatcccaacagagatggagactcatactactattctgagcctacaagtgaaaataatgcccaccacgtctgctggttggaggcctcaatgctcttggacaacatggaggtgaggggtggaatggtcgccccactctatggcgttgaaggaactaaaacaccagtttcccctggtgaaatgagactgagggatgaccagaggaaagtcttcagagaactagtgaggaattgtgacctgcccgtttggctttcgtggcaagtggccaaggctggtttgaagacgaatgatcgtaagtggtgttttgaaggccctgaggaacatgagatcttgaatgacagcggtgaaacagtgaagtgcagggctcctggaggagcaaagaagcctctgcgcccaaggtggtgtgatgaaagggtgtcatctgaccagagtgcgctgtctgaatttattaagtttgctgaaggtaggaggggagctgctgaagtgctagttgtgctgagtgaactccctgatttcctggctaaaaaaggtggagaggcaatggataccatcagtgtgttcctccactctgaggaaggctctagggcttaccgcaatgcactatcaatgatgcctgaggcaatgacaatagtcatgctgtttatactggctggactactgacatcgggaatggtcatctttttcatgtctcccaaaggcatcagtagaatgtctatggcgatgggcacaatggccggctgtggatatctcatgttccttggaggcgtcaaacccactcacatctcctatgtcatgctcatattctttgtcctgatggtggttgtgatccccgagccagggcaacaaaggtccatccaagacaaccaagtggcatacctcattattggcatcctgacgctggtttcagcggtggcagccaacgagctaggcatgctggagaaaaccaaagaggacctctttgggaagaagaacttaattccatctagtgcttcaccctggagttggccggatcttgacctgaagccaggagctgcctggacagtgtacgttggcattgttacaatgctctctccaatgttgcaccactggatcaaagtcgaatatggcaacctgtctctgtctggaatagcccagtcagcctcagtcctttctttcatggacaaggggataccattcatgaagatgaatatctcggtcataatgctgctggtcagtggctggaattcaataacagtgatgcctctgctctgtggcatagggtgcgccatgctccactggtctctcattttacctggaatcaaagcgcagcagtcaaagcttgcacagagaagggtgttccatggcgttgccaagaaccctgtggttgatgggaatccaacagttgacattgaggaagctcctgaaatgcctgccctttatgagaagaaactggctctatatctccttcttgctctcagcctagcttctgttgccatgtgcagaacgcccttttcattggctgaaggcattgtcctagcatcagctgccttagggccgctcatagagggaaacaccagccttctttggaatggacccatggctgtctccatgacaggagtcatgagggggaatcactatgcttttgtgggagtcatgtacaatctatggaagatgaaaactggacgccgggggagcgcgaatggaaaaactttgggtgaagtctggaagagggaactgaatctgttggacaagcgacagtttgagttgtataaaaggaccgacattgtggaggtggatcgtgatacggcacgcaggcatttggccgaagggaaggtggacaccggggtggcggtctccagggggaccgcaaagttaaggtggttccatgagcgtggctatgtcaagctggaaggtagggtgattgacctggggtgtggccgcggaggctggtgttactacgctgctgcgcaaaaggaagtgagtggggtcaaaggatttactcttggaagagacggccatgagaaacccatgaatgtgcaaagtctgggatggaacatcatcaccttcaaggacaaaactgatatccaccgcctagaaccagtgaaatgtgacacccttttgtgtgacattggagagtcatcatcgtcatcggtcacagagggggaaaggaccgtgagagttcttgatactgtagaaaaatggctggcttgtggggttgacaacttctgtgtgaaggtgttagctccatacatgccagatgttcttgagaaactggaattgctccaaaggaggtttggcggaacagtgatcaggaaccctctctccaggaattccactcatgaaatgtactacgtgtctggagcccgcagcaatgtcacatttactgtgaaccaaacatcccgcctcctgatgaggagaatgaggcgtccaactggaaaagtgaccctggaggctgacgtcatcctcccaattgggacacgcagtgttgagacagacaagggacccctggacaaagaggccatagaagaaagggttgagaggataaaatctgagtacatgacctcttggttttatgacaatgacaacccctacaggacctggcactactgtggctcctatgtcacaaaaacctcaggaagtgcggcgagcatggtaaatggtgttattaaaattctgacatatccatgggacaggatagaggaggtcaccagaatggcaatgactgacacaaccccttttggacagcaaagagtgtttaaagaaaaagttgacaccagagcaaaggatccaccagcgggaactaggaagatcatgaaagttgtcaacaggtggctgttccgccacctggccagagaaaagagccccagactgtgcacaaaggaagaatttattgcaaaagtccgaagtcatgcagccattggagcttacctggaagaacaagaacagtggaagactgccaatgaggctgtccaagacccaaagttctgggaactggtggatgaagaaaggaagctgcaccaacaaggcaggtgtcggacttgtgtgtacaacatgatggggaaaagagagaagaagctgtcagagtttgggaaagcaaagggaagccgtgccatatggtatatgtggctgggagcgcggtatcttgagtttgaggccctgggattcctgaatgaggaccattgggcttccagggaaaactcaggaggaggagtggaaggcattggcttacaatacctaggatatgtgatcagagacctggctgcaatggatggtggtggattctacgcggatgacaccgctggatgggacacgcgcatcacagaggcagaccttgatgatgaacaggagatcttgaactacatgagcccacatcacaaaaaactggcacaagcagtgatggaaatgacatacaagaacaaagtggtgaaagtgttgagaccagccccaggagggaaagcctacatggatgtcataagtcgacgagaccagagaggatccgggcaggtagtgacttatgctctgaacaccatcaccaacttgaaagtccaattgatcagaatggcagaagcagagatggtgatacatcaccaacatgttcaagattgtgatgaatcagttctgaccaggctggaggcatggctcactgagcacggatgtaacagactgaagaggatggcggtgagtggagacgactgtgtggtccggcccatcgatgacaggttcggcctggccctgtcccatctcaacgccatgtccaaggttagaaaggacatatctgaatggcagccatcaaaagggtggaatgattgggagaatgtgcccttctgttcccaccacttccatgaactacagctgaaggatggcaggaggattgtggtgccttgccgagaacaggacgagctcattgggagaggaagggtgtctccaggaaacggctggatgatcaaggaaacagcttgcctcagcaaagcctatgccaacatgtggtcactgatgtattttcacaaaagggacatgaggctactgtcattggctgtttcctcagctgttcccacctcatgggttccacaaggacgcacaacatggtcgattcatgggaaaggggagtggatgaccacggaagacatgcttgaggtgtggaacagagtatggataaccaacaacccacacatgcaggacaagacaatggtgaaaaaatggagagatgtcccttatctaaccaagagacaagacaagctgtgcggatcactgattggaatgaccaatagggccacctgggcctcccacatccatttagtcatccatcgtatccgaacgctgattggacaggagaaatacactgactacctaacagtcatggacaggtattctgtggatgctgacctgcaactgggtgagcttatctgaaacaccatctaacaggaataaccgggatacaaaccacgggtggagaaccggactccccacaacctgaaaccgggatataaaccacggctggagaaccgggctccgcacttaaaatgaaacagaaaccgggataaaaactacggatggagaaccggactccacacattgagacagaagaagttgtcagcccagaaccccacacgagttttgccactgctaagctgtgaggcagtgcaggctgggacagccgacctccaggttgcgaaaaacctggtttctgggacctcccaccccagagtaaaaagaacggagcctccgctaccaccctcccacgtggtggtagaaagacggggtctagaggttagaggagaccctccagggaacaaatagtgggaccatattgacgccagggaaagaccggagtggttctctgcttttcctccagaggtctgtgagcacagtttgctcaagaataagcagacctttggatgacaaacacaaaaccac

SEQ ID NO: 6 - protein, 3771 aa, Yellow fever virus
MSGRKAQGKTLGVNMVRRGVRSLSNKIKQKTKQIGNRPGPSRGVQGFIFFFLFNILTGKKITAHLKRLWKMLDPRQGLAVLRKVKRVVASLMRGLSSRKRRSHDVLTVQFLILGMLLMTGGVTLVRKNRWLLLNVTSEDLGKTFSVGTGNCTTNILEAKYWCPDSMEYNCPNLSPREEPDDIDCWCYGVENVRVAYGKCDSAGRSRRSRRAIDLPTHENHGLKTRQEKWMTGRMGERQLQKIERWFVRNPFFAVTALTIAYLVGSNMTQRVVIALLVLAVGPAYSAHCIGITDRDFIEGVHGGTWVSATLEQDKCVTVMAPDKPSLDISLETVAIDRPAEARKVCYNAVLTHVKINDKCPSTGEAHLAEENEGDNACKRTYSDRGWGNGCGLFGKGSIVACAKFTCAKSMSLFEVDQTKIQYVIRAQLHVGAKQENWNTSIKTLKFDALSGSQEVEFIGYGKATLECQVQTAVDFGNSYIAEMETESWIVDRQWAQDLTLPWQSGSGGVWREMHHLVEFEPPHAATIRVLALGNQEGSLKTALTGAMRVTKDTNDNNLYKLHGGHVSCRVKLSALTLKGTSYKICTDKMFFVKNPTDTGHGTVVMQVKVSKGAPCRIPVIVADDLTAAINKGILVTVNPIASTNDDEVLIEVNPPFGDSYIIVGRGDSRLTYQWHKEGSSIGKLFTQTMKGVERLAVMGDTAWDFSSAGGFFTSVGKGIHTVFGSAFQGLFGGLNWITKVIMGAVLIWVGINTRNMTMSMSMILVGVIMMFLSLGVGADQGCAINFGRKGSQTSNTTKWAPPGQGSPGSKGEELFTGVVPILVELDGDVNGHKFSVSGEGEGDATYGKLTLKFICTTGKLPVPWPTLVTTLTYGVQCFSRYPDHMKQHDFFKSAMPEGYVQERTIFFKDDGNYKTRAEVKFEGDTLVNRIELKGIDFKEDGNILGHKLEYNYNSHNVYIMADKQKNGIKVNFKIRHNIEDGSVQLADHYQQNTPIGDGPVLLPDNHYLSTQSALSKDPNEKRDHMVLLEFVTAAGITLGMDELYKGSSPLSHRSKRSLSCRPPMVKEGSSIGTSLGKAVHQVFGSVYTTMFGGVSWMIRILIGFLVLWIGTNSRNTSMAMTCIAVGGITLFLGFTVGADQGCAINFGKRELKCGDGIFIFRDSDDWLNKYSYYPEDPVKLASIVKASFEEGKCGLNSVDSLEHEMWRSRADEINAIFEENEVDISVVVQDPKNVYQRGTHPFSRIRDGLQYGWKTWGKNLVFSPGRKNGSFIIDGKSRKECPFSNRVWNSFQIEEFGTGVFTTRVYMDAVFEYTIDCDGSILGAAVNGKKSAHGSPTFWMGSHEVNGTWMIHTLEALDYKECEWPLTHTIGTSVEESEMFMPRSIGGPVSSHNHIPGYKVQTNGPWMQVPLEVKREACPGTSVIIDGNCDGRGKSTRSTTDSGKVIPEWCCRSCTMPPVSFHGSDGCWYPMEIRPRKTHESHLVRSWVTAGEIHAVPFGLVSMMIAMEVVLRKRQGPKQMLVGGVVLLGAMLVGQVTLLDLLKLTVAVGLHFHEMNNGGDAMYMALIAAFSIRPGLLIGFGLRTLWSPRERLVLTLGAAMVEIALGGVMGGLWKYLNAVSLCILTINAVASRKASNTILPLMALLTPVTMAEVRLAAMFFCAMVIIGVLHQNFKDTSMQKTIPLVALTLTSYLGLTQPFLGLCAFLATRIFGRRSIPVNEALAAAGLVGVLAGLAFQEMENFLGPIAVGGLLMMLVSVAGRVDGLELKKLGEVSWEEEAEISGSSARYDVALSEQGEFKLLSEEKVPWDQVVMTSLALVGAALHPFALLLVLAGWLFHVRGARRSGDVLWDIPTPKIIEECEHLEDGIYGIFQSTFLGASQRGVGVAQGGVFHTMWHVTRGAFLVRNGKKLIPSWASVKEDLVAYGGSWKLEGRWDGEEEVQLIAAVPGKNVVNVQTKPSLFKVRNGGEIGAVALDYPSGTSGSPIVNRNGEVIGLYGNGILVGDNSFVSAISQTEVKEEGKEELQEIPTMLKKGMTTVLDFHPGAGKTRRFLPQILAECARRRLRTLVLAPTRVVLSEMKEAFHGLDVKFHTQAFSAHGSGREVIDAMCHATLTYRMLEPTRVVNWEVIIMDEAHFLDPASIAARGWAAHRARANESATILMTATPPGTSDEFPHSNGEIEDVQTDIPSEPWNTGHDWILADKRPTAWFLPSIRAANVMAASLRKAGKSVVVLNRKTFEREYPTIKQKKPDFILATDIAEMGANLCVERVLDCRTAFKPVLVDEGRKVAIKGPLRISASSAAQRRGRIGRNPNRDGDSYYYSEPTSENNAHHVCWLEASMLLDNMEVRGGMVAPLYGVEGTKTPVSPGEMRLRDDQRKVFRELVRNCDLPVWLSWQVAKAGLKTNDRKWCFEGPEEHEILNDSGETVKCRAPGGAKKPLRPRWCDERVSSDQSALSEFIKFAEGRRGAAEVLVVLSELPDFLAKKGGEAMDTISVFLHSEEGSRAYRNALSMMPEAMTIVMLFILAGLLTSGMVIFFMSPKGISRMSMAMGTMAGCGYLMFLGGVKPTHISYVMLIFFVLMVVVIPEPGQQRSIQDNQVAYLIIGILTLVSAVAANELGMLEKTKEDLFGKKNLIPSSASPWSWPDLDLKPGAAWTVYVGIVTMLSPMLHHWIKVEYGNLSLSGIAQSASVLSFMDKGIPFMKMNISVIMLLVSGWNSITVMPLLCGIGCAMLHWSLILPGIKAQQSKLAQRRVFHGVAKNPVVDGNPTVDIEEAPEMPALYEKKLALYLLLALSLASVAMCRTPFSLAEGIVLASAALGPLIEGNTSLLWNGPMAVSMTGVMRGNHYAFVGVMYNLWKMKTGRRGSANGKTLGEVWKRELNLLDKRQFELYKRTDIVEVDRDTARRHLAEGKVDTGVAVSRGTAKLRWFHERGYVKLEGRVIDLGCGRGGWCYYAAAQKEVSGVKGFTLGRDGHEKPMNVQSLGWNIITFKDKTDIHRLEPVKCDTLLCDIGESSSSSVTEGERTVRVLDTVEKWLACGVDNFCVKVLAPYMPDVLEKLELLQRRFGGTVIRNPLSRNSTHEMYYVSGARSNVTFTVNQTSRLLMRRMRRPTGKVTLEADVILPIGTRSVETDKGPLDKEAIEERVERIKSEYMTSWFYDNDNPYRTWHYCGSYVTKTSGSAASMVNGVIKILTYPWDRIEEVTRMAMTDTTPFGQQRVFKEKVDTRAKDPPAGTRKIMKVVNRWLFRHLAREKSPRLCTKEEFIAKVRSHAAIGAYLEEQEQWKTANEAVQDPKFWELVDEERKLHQQGRCRTCVYNMMGKREKKLSEFGKAKGSRAIWYMWLGARYLEFEALGFLNEDHWASRENSGGGVEGIGLQYLGYVIRDLAAMDGGGFYADDTAGWDTRITEADLDDEQEILNYMSPHHKKLAQAVMEMTYKNKVVKVLRPAPGGKAYMDVISRRDQRGSGQVVTYALNTITNLKVQLIRMAEAEMVIHHQHVQDCDESVLTRLEAWLTEHGCNRLKRMAVSGDDCVVRPIDDRFGLALSHLNAMSKVRKDISEWQPSKGWNDWENVPFCSHHFHELQLKDGRRIVVPCREQDELIGRGRVSPGNGWMIKETACLSKAYANMWSLMYFHKRDMRLLSLAVSSAVPTSWVPQGRTTWSIHGKGEWMTTEDMLEVWNRVWITNNPHMQDKTMVKKWRDVPYLTKRQDKLCGSLIGMTNRATWASHIHLVIHRIRTLIGQEKYTDYLTVMDRYSVDADLQLGELI

SEQ ID NO: 7 - DNA, 12034 bp, Yellow fever virus
agtaaatcctgtgtgctaattgaggtgcattggtctgcaaatcgagttgctaggcaataaacacatttggattaattttaatcgttcgttgagcgattagcagagaactgaccagaacatgtctggtcgtaaagctcagggaaaaaccctgggcgtcaatatggtacgacgaggagttcgctccttgtcaaacaaaataaaacaaaaaacaaaacaaattggaaacagacctggaccttcaagaggtgttcaaggatttatctttttctttttgttcaacattttgactggaaaaaagatcacagcccacctaaagaggttgtggaaaatgctggacccaagacaaggcttggctgttctaaggaaagtcaagagagtggtggccagtttgatgagaggattgtcctcaaggaaacgccgttcccatgatgttctgactgtgcaattcctaattttgggaatgctgttgatgaccggtggagtgaccttggtgcggaaaaacagatggttgctcctaaatgtgacatctgaggacctcgggaaaacattctctgtgggcacaggcaactgcacaacaaacattttggaagccaagtactggtgcccagactcaatggaatacaactgtcccaatctcagtccaagagaggagccagatgacattgattgctggtgctatggggtggaaaacgttagagtcgcatatggtaagtgtgactcagcaggcaggtctaggaggtcaagaagggccattgacttgcctacgcatgaaaaccatggtttgaagacccggcaagaaaaatggatgactggaagaatgggtgaaaggcaactccaaaagattgagagatggttcgtgaggaaccccttttttgcagtgacggctctgaccattgcctaccttgtgggaagcaacatgacgcaacgagtcgtgattgccctactggtcttggctgttggtccggcctactcagctcactgcattggaattactgacagggatttcattgagggggtgcatggaggaacttgggtttcagctaccctggagcaagacaagtgtgtcactgttatggcccctgacaagccttcattggacatctcactagagacagtagccattgatagacctgctgaggcgaggaaagtgtgttacaatgcagttctcactcatgtgaagattaatgacaagtgccccagcactggagaggcccacctagctgaagagaacgaaggggacaatgcgtgcaagcgcacttattctgatagaggctggggcaatggctgtggcctatttgggaaagggagcattgtggcatgcgccaaattcacttgtgccaaatccatgagtttgtttgaggttgatcagaccaaaattcagtatgtcatcagagcacaattgcatgtaggggccaagcaggaaaattggaataccagcattaagactctcaagtttgatgccctgtcaggctcccaggaagtcgagttcattgggtatggaaaagctacactggaatgccaggtgcaaactgcggtggactttggtaacagttacatcgctgagatggaaacagagagctggatagtggacagacagtgggcccaggacttgaccctgccatggcagagtggaagtggcggggtgtggagagagatgcatcatcttgtcgaatttgaacctccgcatgccgccactatcagagtactggccctgggaaaccaggaaggctccttgaaaacagctcttactggcgcaatgagggttacaaaggacacaaatgacaacaacctttacaaactacatggtggacatgtttcttgcagagtgaaattgtcagctttgacactcaaggggacatcctacaaaatatgcactgacaaaatgttttttgtcaagaacccaactgacactggccatggcactgttgtgatgcaggtgaaagtgtcaaaaggagccccctgcaggattccagtgatagtagctgatgatcttacagcggcaatcaataaaggcattttggttacagttaaccccatcgcctcaaccaatgatgatgaagtgctgattgaggtgaacccaccttttggagacagctacattatcgttgggagaggagattcacgtctcacttaccagtggcacaaagagggaagctcaataggaaagttgttcactcagaccatgaaaggcgtggaacgcctggccgtcatgggagacaccgcctgggatttcagctccgctggagggttcttcacttcggttgggaaaggaattcatacggtgtttggctctgcctttcaggggctatttggcggcttgaactggataacaaaggtcatcatgggggcggtacttatatgggttggcatcaacacaagaaacatgacaatgtccatgagcatgatcttggtaggagtgatcatgatgtttttgtctctaggagttggggcggatcaaggatgcgccatcaacttcggccgaaagggatcacaaacctccaacacaactaaatgggctcctcccggacaaggaagtcccgggagcaagggcgaggagctgttcaccggggtggtgcccatcctggtcgagctggacggcgacgtaaacggccacaagttcagcgtgtccggcgagggcgagggcgatgccacctacggcaagctgaccctgaagttcatctgcaccaccggcaagctgcccgtgccctggcccaccctcgtgaccaccctgacctacggcgtgcagtgcttcagccgctaccccgaccacatgaagcagcacgacttcttcaagtccgccatgcccgaaggctacgtccaggagcgcaccatcttcttcaaggacgacggcaactacaagacccgcgccgaggtgaagttcgagggcgacaccctggtgaaccgcatcgagctgaagggcatcgacttcaaggaggacggcaacatcctggggcacaagctggagtacaactacaacagccacaacgtctatatcatggccgacaagcagaagaacggcatcaaggtgaacttcaagatccgccacaacatcgaggacggcagcgtgcagctcgccgaccactaccagcagaacacccccatcggcgacggccccgtgctgctgcccgacaaccactacctgagcacccagtccgccctgagcaaagaccccaacgagaagcgcgatcacatggtcctgctggagttcgtgaccgccgccgggatcactctcggcatggacgagctgtacaagtccggaagcagtccactgtctcatcgcagtaaaaggagcctatcctgtcggccacccatggtcaaagagggaagctcaataggaaagatgtttgagtccacatacagaggtgcaaaacgaatggccattctaggtgaaacagcttgggattttggttccgttggtggactgttcacatcattgggaaaggctgtgcaccaggtttttggaagtgtgtatacaaccatgtttggaggagtctcatggatgattagaatcctaattgggttcttagtgttgtggattggcacgaactccaggaacacttcaatggctatgacgtgcatagctgttggaggaatcactctgtttctgggcttcacagttggcgccgatcaaggatgcgccatcaactttggcaagagagagctcaagtgcggagatggtatcttcatatttagagactctgatgactggctgaacaagtactcatactatccagaagatcctgtgaagcttgcatcaatagtgaaagcctcttttgaagaagggaagtgtggcctaaattcagttgactcccttgagcatgagatgtggagaagcagggcagatgagatcaatgccatttttgaggaaaacgaggtggacatttctgttgtcgtgcaggatccaaagaatgtttaccagagaggaactcatccattttccagaattcgggatggtctgcagtatggttggaagacttggggtaagaaccttgtgttctccccagggaggaagaatggaagcttcatcatagatggaaagtccaggaaagaatgcccgttttcaaaccgggtctggaattctttccagatagaggagtttgggacgggagtgttcaccacacgcgtgtacatggacgcagtctttgaatacaccatagactgcgatggatctatcttgggtgcagcggtgaacggaaaaaagagtgcccatggctctccaacattttggatgggaagtcatgaagtaaatgggacatggatgatccacaccttggaggcattagattacaaggagtgtgagtggccactgacacatacgattggaacatcagttgaagagagtgaaatgttcatgccgagatcaatcggaggcccagttagctctcacaatcatatccctggatacaaggttcagacgaacggaccttggatgcaggtaccactagaagtgaagagagaagcttgcccagggactagcgtgatcattgatggcaactgtgatggacggggaaaatcaaccagatccaccacggatagcgggaaagttattcctgaatggtgttgccgctcctgcacaatgccgcctgtgagcttccatggtagtgatgggtgttggtatcccatggaaattaggccaaggaaaacgcatgaaagccatctggtgcgctcctgggttacagctggagaaatacatgctgtcccttttggtttggtgagcatgatgatagcaatggaagtggtcctaaggaaaagacagggaccaaagcaaatgttggttggaggagtagtgctcttgggagcaatgctggtcgggcaagtaactctccttgatttgctgaaactcacagtggctgtgggattgcatttccatgagatgaacaatggaggagacgccatgtatatggcgttgattgctgccttttcaatcagaccagggctgctcatcggctttgggctcaggaccctatggagccctcgggaacgccttgtgctgaccctaggagcagccatggtggagattgccttgggtggcgtgatgggcggcctgtggaagtatctaaatgcagtttctctctgcatcctgacaataaatgctgttgcttctaggaaagcatcaaataccatcttgcccctcatggctctgttgacacctgtcactatggctgaggtgagacttgccgcaatgttcttttgtgccatggttatcataggggtccttcaccagaatttcaaggacacctccatgcagaagactatacctctggtggccctcacactcacatcttacctgggcttgacacaaccttttttgggcctgtgtgcatttctggcaacccgcatatttgggcgaaggagtatcccagtgaatgaggcactcgcagcagctggtctagtgggagtgctggcaggactggcttttcaggagatggagaacttccttggtccgattgcagttggaggactcctgatgatgctggttagcgtggctgggagggtggatgggctagagctcaagaagcttggtgaagtttcatgggaagaggaggcggagatcagcgggagttccgcccgctatgatgtggcactcagtgaacaaggggagttcaagctgctttctgaagagaaagtgccatgggaccaggttgtgatgacctcgctggccttggttggggctgccctccatccatttgctcttctgctggtccttgctgggtggctgtttcatgtcaggggagctaggagaagtggggatgtcttgtgggatattcccactcctaagatcatcgaggaatgtgaacatctggaggatgggatttatggcatattccagtcaaccttcttgggggcctcccagcgaggagtgggagtggcacagggaggggtgttccacacaatgtggcatgtcacaagaggagctttccttgtcaggaatggcaagaagttgattccatcttgggcttcagtaaaggaagaccttgtcgcctatggtggctcatggaagttggaaggcagatgggatggagaggaagaggtccagttgatcgcggctgttccaggaaagaacgtggtcaacgtccagacaaaaccgagcttgttcaaagtgaggaatgggggagaaatcggggctgtcgctcttgactatccgagtggcacttcaggatctcctattgttaacaggaacggagaggtgattgggctgtacggcaatggcatccttgtcggtgacaactccttcgtgtccgccatatcccagactgaggtgaaggaagaaggaaaggaggagctccaagagatcccgacaatgctaaagaaaggaatgacaactgtccttgattttcatcctggagctgggaagacaagacgtttcctcccacagatcttggccgagtgcgcacggagacgcttgcgcactcttgtgttggcccccaccagggttgttctttctgaaatgaaggaggcttttcacggcctggacgtgaaattccacacacaggctttttccgctcacggcagcgggagagaagtcattgatgccatgtgccatgccaccctaacttacaggatgttggaaccaactagggttgttaactgggaagtgatcattatggatgaagcccattttttggatccagctagcatagccgctagaggttgggcagcgcacagagctagggcaaatgaaagtgcaacaatcttgatgacagccacaccgcctgggactagtgatgaatttccacattcaaatggtgaaatagaagatgttcaaacggacatacccagtgagccctggaacacagggcatgactggatcctggctgacaaaaggcccacggcatggttccttccatccatcagagctgcaaatgtcatggctgcctctttgcgtaaggctggaaagagtgtggtggtcctgaacaggaaaacctttgagagagaataccccacgataaagcagaagaaacctgactttatattggccactgacatagctgaaatgggagccaacctttgcgtggagcgagtgctggattgcaggacggcttttaagcctgtgcttgtggatgaagggaggaaggtggcaataaaagggccacttcgtatctccgcatcctctgctgctcaaaggagggggcgcattgggagaaatcccaacagagatggagactcatactactattctgagcctacaagtgaaaataatgcccaccacgtctgctggttggaggcctcaatgctcttggacaacatggaggtgaggggtggaatggtcgccccactctatggcgttgaaggaactaaaacaccagtttcccctggtgaaatgagactgagggatgaccagaggaaagtcttcagagaactagtgaggaattgtgacctgcccgtttggctttcgtggcaagtggccaaggctggtttgaagacgaatgatcgtaagtggtgttttgaaggccctgaggaacatgagatcttgaatgacagcggtgaaacagtgaagtgcagggctcctggaggagcaaagaagcctctgcgcccaaggtggtgtgatgaaagggtgtcatctgaccagagtgcgctgtctgaatttattaagtttgctgaaggtaggaggggagctgctgaagtgctagttgtgctgagtgaactccctgatttcctggctaaaaaaggtggagaggcaatggataccatcagtgtgttcctccactctgaggaaggctctagggcttaccgcaatgcactatcaatgatgcctgaggcaatgacaatagtcatgctgtttatactggctggactactgacatcgggaatggtcatctttttcatgtctcccaaaggcatcagtagaatgtctatggcgatgggcacaatggccggctgtggatatctcatgttccttggaggcgtcaaacccactcacatctcctatgtcatgctcatattctttgtcctgatggtggttgtgatccccgagccagggcaacaaaggtccatccaagacaaccaagtggcatacctcattattggcatcctgacgctggtttcagcggtggcagccaacgagctaggcatgctggagaaaaccaaagaggacctctttgggaagaagaacttaattccatctagtgcttcaccctggagttggccggatcttgacctgaagccaggagctgcctggacagtgtacgttggcattgttacaatgctctctccaatgttgcaccactggatcaaagtcgaatatggcaacctgtctctgtctggaatagcccagtcagcctcagtcctttctttcatggacaaggggataccattcatgaagatgaatatctcggtcataatgctgctggtcagtggctggaattcaataacagtgatgcctctgctctgtggcatagggtgcgccatgctccactggtctctcattttacctggaatcaaagcgcagcagtcaaagcttgcacagagaagggtgttccatggcgttgccaagaaccctgtggttgatgggaatccaacagttgacattgaggaagctcctgaaatgcctgccctttatgagaagaaactggctctatatctccttcttgctctcagcctagcttctgttgccatgtgcagaacgcccttttcattggctgaaggcattgtcctagcatcagctgccttagggccgctcatagagggaaacaccagccttctttggaatggacccatggctgtctccatgacaggagtcatgagggggaatcactatgcttttgtgggagtcatgtacaatctatggaagatgaaaactggacgccgggggagcgcgaatggaaaaactttgggtgaagtctggaagagggaactgaatctgttggacaagcgacagtttgagttgtataaaaggaccgacattgtggaggtggatcgtgatacggcacgcaggcatttggccgaagggaaggtggacaccggggtggcggtctccagggggaccgcaaagttaaggtggttccatgagcgtggctatgtcaagctggaaggtagggtgattgacctggggtgtggccgcggaggctggtgttactacgctgctgcgcaaaaggaagtgagtggggtcaaaggatttactcttggaagagacggccatgagaaacccatgaatgtgcaaagtctgggatggaacatcatcaccttcaaggacaaaactgatatccaccgcctagaaccagtgaaatgtgacacccttttgtgtgacattggagagtcatcatcgtcatcggtcacagagggggaaaggaccgtgagagttcttgatactgtagaaaaatggctggcttgtggggttgacaacttctgtgtgaaggtgttagctccatacatgccagatgttcttgagaaactggaattgctccaaaggaggtttggcggaacagtgatcaggaaccctctctccaggaattccactcatgaaatgtactacgtgtctggagcccgcagcaatgtcacatttactgtgaaccaaacatcccgcctcctgatgaggagaatgaggcgtccaactggaaaagtgaccctggaggctgacgtcatcctcccaattgggacacgcagtgttgagacagacaagggacccctggacaaagaggccatagaagaaagggttgagaggataaaatctgagtacatgacctcttggttttatgacaatgacaacccctacaggacctggcactactgtggctcctatgtcacaaaaacctcaggaagtgcggcgagcatggtaaatggtgttattaaaattctgacatatccatgggacaggatagaggaggtcaccagaatggcaatgactgacacaaccccttttggacagcaaagagtgtttaaagaaaaagttgacaccagagcaaaggatccaccagcgggaactaggaagatcatgaaagttgtcaacaggtggctgttccgccacctggccagagaaaagagccccagactgtgcacaaaggaagaatttattgcaaaagtccgaagtcatgcagccattggagcttacctggaagaacaagaacagtggaagactgccaatgaggctgtccaagacccaaagttctgggaactggtggatgaagaaaggaagctgcaccaacaaggcaggtgtcggacttgtgtgtacaacatgatggggaaaagagagaagaagctgtcagagtttgggaaagcaaagggaagccgtgccatatggtatatgtggctgggagcgcggtatcttgagtttgaggccctgggattcctgaatgaggaccattgggcttccagggaaaactcaggaggaggagtggaaggcattggcttacaatacctaggatatgtgatcagagacctggctgcaatggatggtggtggattctacgcggatgacaccgctggatgggacacgcgcatcacagaggcagaccttgatgatgaacaggagatcttgaactacatgagcccacatcacaaaaaactggcacaagcagtgatggaaatgacatacaagaacaaagtggtgaaagtgttgagaccagccccaggagggaaagcctacatggatgtcataagtcgacgagaccagagaggatccgggcaggtagtgacttatgctctgaacaccatcaccaacttgaaagtccaattgatcagaatggcagaagcagagatggtgatacatcaccaacatgttcaagattgtgatgaatcagttctgaccaggctggaggcatggctcactgagcacggatgtaacagactgaagaggatggcggtgagtggagacgactgtgtggtccggcccatcgatgacaggttcggcctggccctgtcccatctcaacgccatgtccaaggttagaaaggacatatctgaatggcagccatcaaaagggtggaatgattgggagaatgtgcccttctgttcccaccacttccatgaactacagctgaaggatggcaggaggattgtggtgccttgccgagaacaggacgagctcattgggagaggaagggtgtctccaggaaacggctggatgatcaaggaaacagcttgcctcagcaaagcctatgccaacatgtggtcactgatgtattttcacaaaagggacatgaggctactgtcattggctgtttcctcagctgttcccacctcatgggttccacaaggacgcacaacatggtcgattcatgggaaaggggagtggatgaccacggaagacatgcttgaggtgtggaacagagtatggataaccaacaacccacacatgcaggacaagacaatggtgaaaaaatggagagatgtcccttatctaaccaagagacaagacaagctgtgcggatcactgattggaatgaccaatagggccacctgggcctcccacatccatttagtcatccatcgtatccgaacgctgattggacaggagaaatacactgactacctaacagtcatggacaggtattctgtggatgctgacctgcaactgggtgagcttatctgaaacaccatctaacaggaataaccgggatacaaaccacgggtggagaaccggactccccacaacctgaaaccgggatataaaccacggctggagaaccgggctccgcacttaaaatgaaacagaaaccgggataaaaactacggatggagaaccggactccacacattgagacagaagaagttgtcagcccagaaccccacacgagttttgccactgctaagctgtgaggcagtgcaggctgggacagccgacctccaggttgcgaaaaacctggtttctgggacctcccaccccagagtaaaaagaacggagcctccgctaccaccctcccacgtggtggtagaaagacggggtctagaggttagaggagaccctccagggaacaaatagtgggaccatattgacgccagggaaagaccggagtggttctctgcttttcctccagaggtctgtgagcacagtttgctcaagaataagcagacctttggatgacaaacacaaaaccac

SEQ ID NO: 8 - protein, 3802 aa, Yellow fever virus
MSGRKAQGKTLGVNMVRRGVRSLSNKIKQKTKQIGNRPGPSRGVQGFIFFFLFNILTGKKITAHLKRLWKMLDPRQGLAVLRKVKRVVASLMRGLSSRKRRSHDVLTVQFLILGMLLMTGGVTLVRKNRWLLLNVTSEDLGKTFSVGTGNCTTNILEAKYWCPDSMEYNCPNLSPREEPDDIDCWCYGVENVRVAYGKCDSAGRSRRSRRAIDLPTHENHGLKTRQEKWMTGRMGERQLQKIERWFVRNPFFAVTALTIAYLVGSNMTQRVVIALLVLAVGPAYSAHCIGITDRDFIEGVHGGTWVSATLEQDKCVTVMAPDKPSLDISLETVAIDRPAEARKVCYNAVLTHVKINDKCPSTGEAHLAEENEGDNACKRTYSDRGWGNGCGLFGKGSIVACAKFTCAKSMSLFEVDQTKIQYVIRAQLHVGAKQENWNTSIKTLKFDALSGSQEVEFIGYGKATLECQVQTAVDFGNSYIAEMETESWIVDRQWAQDLTLPWQSGSGGVWREMHHLVEFEPPHAATIRVLALGNQEGSLKTALTGAMRVTKDTNDNNLYKLHGGHVSCRVKLSALTLKGTSYKICTDKMFFVKNPTDTGHGTVVMQVKVSKGAPCRIPVIVADDLTAAINKGILVTVNPIASTNDDEVLIEVNPPFGDSYIIVGRGDSRLTYQWHKEGSSIGKLFTQTMKGVERLAVMGDTAWDFSSAGGFFTSVGKGIHTVFGSAFQGLFGGLNWITKVIMGAVLIWVGINTRNMTMSMSMILVGVIMMFLSLGVGADQGCAINFGRKGSQTSNTTKWAPPGQGSPGSKGEELFTGVVPILVELDGDVNGHKFSVSGEGEGDATYGKLTLKFICTTGKLPVPWPTLVTTLTYGVQCFSRYPDHMKQHDFFKSAMPEGYVQERTIFFKDDGNYKTRAEVKFEGDTLVNRIELKGIDFKEDGNILGHKLEYNYNSHNVYIMADKQKNGIKVNFKIRHNIEDGSVQLADHYQQNTPIGDGPVLLPDNHYLSTQSALSKDPNEKRDHMVLLEFVTAAGITLGMDELYKSGSSPLSHRSKRSLSCRPPMVKEGSSIGKMFESTYRGAKRMAILGETAWDFGSVGGLFTSLGKAVHQVFGSVYTTMFGGVSWMIRILIGFLVLWIGTNSRNTSMAMTCIAVGGITLFLGFTVGADQGCAINFGKRELKCGDGIFIFRDSDDWLNKYSYYPEDPVKLASIVKASFEEGKCGLNSVDSLEHEMWRSRADEINAIFEENEVDISVVVQDPKNVYQRGTHPFSRIRDGLQYGWKTWGKNLVFSPGRKNGSFIIDGKSRKECPFSNRVWNSFQIEEFGTGVFTTRVYMDAVFEYTIDCDGSILGAAVNGKKSAHGSPTFWMGSHEVNGTWMIHTLEALDYKECEWPLTHTIGTSVEESEMFMPRSIGGPVSSHNHIPGYKVQTNGPWMQVPLEVKREACPGTSVIIDGNCDGRGKSTRSTTDSGKVIPEWCCRSCTMPPVSFHGSDGCWYPMEIRPRKTHESHLVRSWVTAGEIHAVPFGLVSMMIAMEVVLRKRQGPKQMLVGGVVLLGAMLVGQVTLLDLLKLTVAVGLHFHEMNNGGDAMYMALIAAFSIRPGLLIGFGLRTLWSPRERLVLTLGAAMVEIALGGVMGGLWKYLNAVSLCILTINAVASRKASNTILPLMALLTPVTMAEVRLAAMFFCAMVIIGVLHQNFKDTSMQKTIPLVALTLTSYLGLTQPFLGLCAFLATRIFGRRSIPVNEALAAAGLVGVLAGLAFQEMENFLGPIAVGGLLMMLVSVAGRVDGLELKKLGEVSWEEEAEISGSSARYDVALSEQGEFKLLSEEKVPWDQVVMTSLALVGAALHPFALLLVLAGWLFHVRGARRSGDVLWDIPTPKIIEECEHLEDGIYGIFQSTFLGASQRGVGVAQGGVFHTMWHVTRGAFLVRNGKKLIPSWASVKEDLVAYGGSWKLEGRWDGEEEVQLIAAVPGKNVVNVQTKPSLFKVRNGGEIGAVALDYPSGTSGSPIVNRNGEVIGLYGNGILVGDNSFVSAISQTEVKEEGKEELQEIPTMLKKGMTTVLDFHPGAGKTRRFLPQILAECARRRLRTLVLAPTRVVLSEMKEAFHGLDVKFHTQAFSAHGSGREVIDAMCHATLTYRMLEPTRVVNWEVIIMDEAHFLDPASIAARGWAAHRARANESATILMTATPPGTSDEFPHSNGEIEDVQTDIPSEPWNTGHDWILADKRPTAWFLPSIRAANVMAASLRKAGKSVVVLNRKTFEREYPTIKQKKPDFILATDIAEMGANLCVERVLDCRTAFKPVLVDEGRKVAIKGPLRISASSAAQRRGRIGRNPNRDGDSYYYSEPTSENNAHHVCWLEASMLLDNMEVRGGMVAPLYGVEGTKTPVSPGEMRLRDDQRKVFRELVRNCDLPVWLSWQVAKAGLKTNDRKWCFEGPEEHEILNDSGETVKCRAPGGAKKPLRPRWCDERVSSDQSALSEFIKFAEGRRGAAEVLVVLSELPDFLAKKGGEAMDTISVFLHSEEGSRAYRNALSMMPEAMTIVMLFILAGLLTSGMVIFFMSPKGISRMSMAMGTMAGCGYLMFLGGVKPTHISYVMLIFFVLMVVVIPEPGQQRSIQDNQVAYLIIGILTLVSAVAANELGMLEKTKEDLFGKKNLIPSSASPWSWPDLDLKPGAAWTVYVGIVTMLSPMLHHWIKVEYGNLSLSGIAQSASVLSFMDKGIPFMKMNISVIMLLVSGWNSITVMPLLCGIGCAMLHWSLILPGIKAQQSKLAQRRVFHGVAKNPVVDGNPTVDIEEAPEMPALYEKKLALYLLLALSLASVAMCRTPFSLAEGIVLASAALGPLIEGNTSLLWNGPMAVSMTGVMRGNHYAFVGVMYNLWKMKTGRRGSANGKTLGEVWKRELNLLDKRQFELYKRTDIVEVDRDTARRHLAEGKVDTGVAVSRGTAKLRWFHERGYVKLEGRVIDLGCGRGGWCYYAAAQKEVSGVKGFTLGRDGHEKPMNVQSLGWNIITFKDKTDIHRLEPVKCDTLLCDIGESSSSSVTEGERTVRVLDTVEKWLACGVDNFCVKVLAPYMPDVLEKLELLQRRFGGTVIRNPLSRNSTHEMYYVSGARSNVTFTVNQTSRLLMRRMRRPTGKVTLEADVILPIGTRSVETDKGPLDKEAIEERVERIKSEYMTSWFYDNDNPYRTWHYCGSYVTKTSGSAASMVNGVIKILTYPWDRIEEVTRMAMTDTTPFGQQRVFKEKVDTRAKDPPAGTRKIMKVVNRWLFRHLAREKSPRLCTKEEFIAKVRSHAAIGAYLEEQEQWKTANEAVQDPKFWELVDEERKLHQQGRCRTCVYNMMGKREKKLSEFGKAKGSRAIWYMWLGARYLEFEALGFLNEDHWASRENSGGGVEGIGLQYLGYVIRDLAAMDGGGFYADDTAGWDTRITEADLDDEQEILNYMSPHHKKLAQAVMEMTYKNKVVKVLRPAPGGKAYMDVISRRDQRGSGQVVTYALNTITNLKVQLIRMAEAEMVIHHQHVQDCDESVLTRLEAWLTEHGCNRLKRMAVSGDDCVVRPIDDRFGLALSHLNAMSKVRKDISEWQPSKGWNDWENVPFCSHHFHELQLKDGRRIVVPCREQDELIGRGRVSPGNGWMIKETACLSKAYANMWSLMYFHKRDMRLLSLAVSSAVPTSWVPQGRTTWSIHGKGEWMTTEDMLEVWNRVWITNNPHMQDKTMVKKWRDVPYLTKRQDKLCGSLIGMTNRATWASHIHLVIHRIRTLIGQEKYTDYLTVMDRYSVDADLQLGELI

SEQ ID NO: 9 - DNA, 11929 bp, Yellow fever virus
agtaaatcctgtgtgctaattgaggtgcattggtctgcaaatcgagttgctaggcaataaacacatttggattaattttaatcgttcgttgagcgattagcagagaactgaccagaacatgtctggtcgtaaagctcagggaaaaaccctgggcgtcaatatggtacgacgaggagttcgctccttgtcaaacaaaataaaacaaaaaacaaaacaaattggaaacagacctggaccttcaagaggtgttcaaggatttatctttttctttttgttcaacattttgactggaaaaaagatcacagcccacctaaagaggttgtggaaaatgctggacccaagacaaggcttggctgttctaaggaaagtcaagagagtggtggccagtttgatgagaggattgtcctcaaggaaacgccgttcccatgatgttctgactgtgcaattcctaattttgggaatgctgttgatgaccggtggagtgaccttggtgcggaaaaacagatggttgctcctaaatgtgacatctgaggacctcgggaaaacattctctgtgggcacaggcaactgcacaacaaacattttggaagccaagtactggtgcccagactcaatggaatacaactgtcccaatctcagtccaagagaggagccagatgacattgattgctggtgctatggggtggaaaacgttagagtcgcatatggtaagtgtgactcagcaggcaggtctaggaggtcaagaagggccattgacttgcctacgcatgaaaaccatggtttgaagacccggcaagaaaaatggatgactggaagaatgggtgaaaggcaactccaaaagattgagagatggttcgtgaggaaccccttttttgcagtgacggctctgaccattgcctaccttgtgggaagcaacatgacgcaacgagtcgtgattgccctactggtcttggctgttggtccggcctactcagctcactgcattggaattactgacagggatttcattgagggggtgcatggaggaacttgggtttcagctaccctggagcaagacaagtgtgtcactgttatggcccctgacaagccttcattggacatctcactagagacagtagccattgatagacctgctgaggcgaggaaagtgtgttacaatgcagttctcactcatgtgaagattaatgacaagtgccccagcactggagaggcccacctagctgaagagaacgaaggggacaatgcgtgcaagcgcacttattctgatagaggctggggcaatggctgtggcctatttgggaaagggagcattgtggcatgcgccaaattcacttgtgccaaatccatgagtttgtttgaggttgatcagaccaaaattcagtatgtcatcagagcacaattgcatgtaggggccaagcaggaaaattggaataccagcattaagactctcaagtttgatgccctgtcaggctcccaggaagtcgagttcattgggtatggaaaagctacactggaatgccaggtgcaaactgcggtggactttggtaacagttacatcgctgagatggaaacagagagctggatagtggacagacagtgggcccaggacttgaccctgccatggcagagtggaagtggcggggtgtggagagagatgcatcatcttgtcgaatttgaacctccgcatgccgccactatcagagtactggccctgggaaaccaggaaggctccttgaaaacagctcttactggcgcaatgagggttacaaaggacacaaatgacaacaacctttacaaactacatggtggacatgtttcttgcagagtgaaattgtcagctttgacactcaaggggacatcctacaaaatatgcactgacaaaatgttttttgtcaagaacccaactgacactggccatggcactgttgtgatgcaggtgaaagtgtcaaaaggagccccctgcaggattccagtgatagtagctgatgatcttacagcggcaatcaataaaggcattttggttacagttaaccccatcgcctcaaccaatgatgatgaagtgctgattgaggtgaacccaccttttggagacagctacattatcgttgggagaggagattcacgtctcacttaccagtggcacaaagagggaagctcaataggaaagttgttcactcagaccatgaaaggcgtggaacgcctggccgtcatgggagacaccgcctgggatttcagctccgctggagggttcttcacttcggttgggaaaggaattcatacggtgtttggctctgcctttcaggggctatttggcggcttgaactggataacaaaggtcatcatgggggcggtacttatatgggttggcatcaacacaagaaacatgacaatgtccatgagcatgatcttggtaggagtgatcatgatgtttttgtctctaggagttggggcggatcaaggatgcgccatcaacttcggccgaaagtcaggggaagaacatgcagtcggaaatactacaggaagtagcaagggcgaggagctgttcaccggggtggtgcccatcctggtcgagctggacggcgacgtaaacggccacaagttcagcgtgtccggcgagggcgagggcgatgccacctacggcaagctgaccctgaagttcatctgcaccaccggcaagctgcccgtgccctggcccaccctcgtgaccaccctgacctacggcgtgcagtgcttcagccgctaccccgaccacatgaagcagcacgacttcttcaagtccgccatgcccgaaggctacgtccaggagcgcaccatcttcttcaaggacgacggcaactacaagacccgcgccgaggtgaagttcgagggcgacaccctggtgaaccgcatcgagctgaagggcatcgacttcaaggaggacggcaacatcctggggcacaagctggagtacaactacaacagccacaacgtctatatcatggccgacaagcagaagaacggcatcaaggtgaacttcaagatccgccacaacatcgaggacggcagcgtgcagctcgccgaccactaccagcagaacacccccatcggcgacggccccgtgctgctgcccgacaaccactacctgagcacccagtccgccctgagcaaagaccccaacgagaagcgcgatcacatggtcctgctggagttcgtgaccgccgccgggatcactctcggcatggacgagctgtacaagagtggagggaaacaggaaggctcacggacaaggcgctcagtgctgatcccatcccatgctcagggaaaagagggaagctcaataggaacatcattgggaaaggctgtgcaccaggtttttggaagtgtgtatacaaccatgtttggaggagtctcatggatgattagaatcctaattgggttcttagtgttgtggattggcacgaactcaaggaacacttcaatggctatgacgtgcatagctgttggaggaatcactctgtttctgggcttcacagttggcgccgatcaaggatgcgccatcaactttggcaagagagagctcaagtgcggagatggtatcttcatatttagagactctgatgactggctgaacaagtactcatactatccagaagatcctgtgaagcttgcatcaatagtgaaagcctcttttgaagaagggaagtgtggcctaaattcagttgactcccttgagcatgagatgtggagaagcagggcagatgagatcaatgccatttttgaggaaaacgaggtggacatttctgttgtcgtgcaggatccaaagaatgtttaccagagaggaactcatccattttccagaattcgggatggtctgcagtatggttggaagacttggggtaagaaccttgtgttctccccagggaggaagaatggaagcttcatcatagatggaaagtccaggaaagaatgcccgttttcaaaccgggtctggaattctttccagatagaggagtttgggacgggagtgttcaccacacgcgtgtacatggacgcagtctttgaatacaccatagactgcgatggatctatcttgggtgcagcggtgaacggaaaaaagagtgcccatggctctccaacattttggatgggaagtcatgaagtaaatgggacatggatgatccacaccttggaggcattagattacaaggagtgtgagtggccactgacacatacgattggaacatcagttgaagagagtgaaatgttcatgccgagatcaatcggaggcccagttagctctcacaatcatatccctggatacaaggttcagacgaacggaccttggatgcaggtaccactagaagtgaagagagaagcttgcccagggactagcgtgatcattgatggcaactgtgatggacggggaaaatcaaccagatccaccacggatagcgggaaagttattcctgaatggtgttgccgctcctgcacaatgccgcctgtgagcttccatggtagtgatgggtgttggtatcccatggaaattaggccaaggaaaacgcatgaaagccatctggtgcgctcctgggttacagctggagaaatacatgctgtcccttttggtttggtgagcatgatgatagcaatggaagtggtcctaaggaaaagacagggaccaaagcaaatgttggttggaggagtagtgctcttgggagcaatgctggtcgggcaagtaactctccttgatttgctgaaactcacagtggctgtgggattgcatttccatgagatgaacaatggaggagacgccatgtatatggcgttgattgctgccttttcaatcagaccagggctgctcatcggctttgggctcaggaccctatggagccctcgggaacgccttgtgctgaccctaggagcagccatggtggagattgccttgggtggcgtgatgggcggcctgtggaagtatctaaatgcagtttctctctgcatcctgacaataaatgctgttgcttctaggaaagcatcaaataccatcttgcccctcatggctctgttgacacctgtcactatggctgaggtgagacttgccgcaatgttcttttgtgccatggttatcataggggtccttcaccagaatttcaaggacacctccatgcagaagactatacctctggtggccctcacactcacatcttacctgggcttgacacaaccttttttgggcctgtgtgcatttctggcaacccgcatatttgggcgaaggagtatcccagtgaatgaggcactcgcagcagctggtctagtgggagtgctggcaggactggcttttcaggagatggagaacttccttggtccgattgcagttggaggactcctgatgatgctggttagcgtggctgggagggtggatgggctagagctcaagaagcttggtgaagtttcatgggaagaggaggcggagatcagcgggagttccgcccgctatgatgtggcactcagtgaacaaggggagttcaagctgctttctgaagagaaagtgccatgggaccaggttgtgatgacctcgctggccttggttggggctgccctccatccatttgctcttctgctggtccttgctgggtggctgtttcatgtcaggggagctaggagaagtggggatgtcttgtgggatattcccactcctaagatcatcgaggaatgtgaacatctggaggatgggatttatggcatattccagtcaaccttcttgggggcctcccagcgaggagtgggagtggcacagggaggggtgttccacacaatgtggcatgtcacaagaggagctttccttgtcaggaatggcaagaagttgattccatcttgggcttcagtaaaggaagaccttgtcgcctatggtggctcatggaagttggaaggcagatgggatggagaggaagaggtccagttgatcgcggctgttccaggaaagaacgtggtcaacgtccagacaaaaccgagcttgttcaaagtgaggaatgggggagaaatcggggctgtcgctcttgactatccgagtggcacttcaggatctcctattgttaacaggaacggagaggtgattgggctgtacggcaatggcatccttgtcggtgacaactccttcgtgtccgccatatcccagactgaggtgaaggaagaaggaaaggaggagctccaagagatcccgacaatgctaaagaaaggaatgacaactgtccttgattttcatcctggagctgggaagacaagacgtttcctcccacagatcttggccgagtgcgcacggagacgcttgcgcactcttgtgttggcccccaccagggttgttctttctgaaatgaaggaggcttttcacggcctggacgtgaaattccacacacaggctttttccgctcacggcagcgggagagaagtcattgatgccatgtgccatgccaccctaacttacaggatgttggaaccaactagggttgttaactgggaagtgatcattatggatgaagcccattttttggatccagctagcatagccgctagaggttgggcagcgcacagagctagggcaaatgaaagtgcaacaatcttgatgacagccacaccgcctgggactagtgatgaatttccacattcaaatggtgaaatagaagatgttcaaacggacatacccagtgagccctggaacacagggcatgactggatcctggctgacaaaaggcccacggcatggttccttccatccatcagagctgcaaatgtcatggctgcctctttgcgtaaggctggaaagagtgtggtggtcctgaacaggaaaacctttgagagagaataccccacgataaagcagaagaaacctgactttatattggccactgacatagctgaaatgggagccaacctttgcgtggagcgagtgctggattgcaggacggcttttaagcctgtgcttgtggatgaagggaggaaggtggcaataaaagggccacttcgtatctccgcatcctctgctgctcaaaggagggggcgcattgggagaaatcccaacagagatggagactcatactactattctgagcctacaagtgaaaataatgcccaccacgtctgctggttggaggcctcaatgctcttggacaacatggaggtgaggggtggaatggtcgccccactctatggcgttgaaggaactaaaacaccagtttcccctggtgaaatgagactgagggatgaccagaggaaagtcttcagagaactagtgaggaattgtgacctgcccgtttggctttcgtggcaagtggccaaggctggtttgaagacgaatgatcgtaagtggtgttttgaaggccctgaggaacatgagatcttgaatgacagcggtgaaacagtgaagtgcagggctcctggaggagcaaagaagcctctgcgcccaaggtggtgtgatgaaagggtgtcatctgaccagagtgcgctgtctgaatttattaagtttgctgaaggtaggaggggagctgctgaagtgctagttgtgctgagtgaactccctgatttcctggctaaaaaaggtggagaggcaatggataccatcagtgtgttcctccactctgaggaaggctctagggcttaccgcaatgcactatcaatgatgcctgaggcaatgacaatagtcatgctgtttatactggctggactactgacatcgggaatggtcatctttttcatgtctcccaaaggcatcagtagaatgtctatggcgatgggcacaatggccggctgtggatatctcatgttccttggaggcgtcaaacccactcacatctcctatgtcatgctcatattctttgtcctgatggtggttgtgatccccgagccagggcaacaaaggtccatccaagacaaccaagtggcatacctcattattggcatcctgacgctggtttcagcggtggcagccaacgagctaggcatgctggagaaaaccaaagaggacctctttgggaagaagaacttaattccatctagtgcttcaccctggagttggccggatcttgacctgaagccaggagctgcctggacagtgtacgttggcattgttacaatgctctctccaatgttgcaccactggatcaaagtcgaatatggcaacctgtctctgtctggaatagcccagtcagcctcagtcctttctttcatggacaaggggataccattcatgaagatgaatatctcggtcataatgctgctggtcagtggctggaattcaataacagtgatgcctctgctctgtggcatagggtgcgccatgctccactggtctctcattttacctggaatcaaagcgcagcagtcaaagcttgcacagagaagggtgttccatggcgttgccaagaaccctgtggttgatgggaatccaacagttgacattgaggaagctcctgaaatgcctgccctttatgagaagaaactggctctatatctccttcttgctctcagcctagcttctgttgccatgtgcagaacgcccttttcattggctgaaggcattgtcctagcatcagctgccttagggccgctcatagagggaaacaccagccttctttggaatggacccatggctgtctccatgacaggagtcatgagggggaatcactatgcttttgtgggagtcatgtacaatctatggaagatgaaaactggacgccgggggagcgcgaatggaaaaactttgggtgaagtctggaagagggaactgaatctgttggacaagcgacagtttgagttgtataaaaggaccgacattgtggaggtggatcgtgatacggcacgcaggcatttggccgaagggaaggtggacaccggggtggcggtctccagggggaccgcaaagttaaggtggttccatgagcgtggctatgtcaagctggaaggtagggtgattgacctggggtgtggccgcggaggctggtgttactacgctgctgcgcaaaaggaagtgagtggggtcaaaggatttactcttggaagagacggccatgagaaacccatgaatgtgcaaagtctgggatggaacatcatcaccttcaaggacaaaactgatatccaccgcctagaaccagtgaaatgtgacacccttttgtgtgacattggagagtcatcatcgtcatcggtcacagagggggaaaggaccgtgagagttcttgatactgtagaaaaatggctggcttgtggggttgacaacttctgtgtgaaggtgttagctccatacatgccagatgttcttgagaaactggaattgctccaaaggaggtttggcggaacagtgatcaggaaccctctctccaggaattccactcatgaaatgtactacgtgtctggagcccgcagcaatgtcacatttactgtgaaccaaacatcccgcctcctgatgaggagaatgaggcgtccaactggaaaagtgaccctggaggctgacgtcatcctcccaattgggacacgcagtgttgagacagacaagggacccctggacaaagaggccatagaagaaagggttgagaggataaaatctgagtacatgacctcttggttttatgacaatgacaacccctacaggacctggcactactgtggctcctatgtcacaaaaacctcaggaagtgcggcgagcatggtaaatggtgttattaaaattctgacatatccatgggacaggatagaggaggtcaccagaatggcaatgactgacacaaccccttttggacagcaaagagtgtttaaagaaaaagttgacaccagagcaaaggatccaccagcgggaactaggaagatcatgaaagttgtcaacaggtggctgttccgccacctggccagagaaaagagccccagactgtgcacaaaggaagaatttattgcaaaagtccgaagtcatgcagccattggagcttacctggaagaacaagaacagtggaagactgccaatgaggctgtccaagacccaaagttctgggaactggtggatgaagaaaggaagctgcaccaacaaggcaggtgtcggacttgtgtgtacaacatgatggggaaaagagagaagaagctgtcagagtttgggaaagcaaagggaagccgtgccatatggtatatgtggctgggagcgcggtatcttgagtttgaggccctgggattcctgaatgaggaccattgggcttccagggaaaactcaggaggaggagtggaaggcattggcttacaatacctaggatatgtgatcagagacctggctgcaatggatggtggtggattctacgcggatgacaccgctggatgggacacgcgcatcacagaggcagaccttgatgatgaacaggagatcttgaactacatgagcccacatcacaaaaaactggcacaagcagtgatggaaatgacatacaagaacaaagtggtgaaagtgttgagaccagccccaggagggaaagcctacatggatgtcataagtcgacgagaccagagaggatccgggcaggtagtgacttatgctctgaacaccatcaccaacttgaaagtccaattgatcagaatggcagaagcagagatggtgatacatcaccaacatgttcaagattgtgatgaatcagttctgaccaggctggaggcatggctcactgagcacggatgtaacagactgaagaggatggcggtgagtggagacgactgtgtggtccggcccatcgatgacaggttcggcctggccctgtcccatctcaacgccatgtccaaggttagaaaggacatatctgaatggcagccatcaaaagggtggaatgattgggagaatgtgcccttctgttcccaccacttccatgaactacagctgaaggatggcaggaggattgtggtgccttgccgagaacaggacgagctcattgggagaggaagggtgtctccaggaaacggctggatgatcaaggaaacagcttgcctcagcaaagcctatgccaacatgtggtcactgatgtattttcacaaaagggacatgaggctactgtcattggctgtttcctcagctgttcccacctcatgggttccacaaggacgcacaacatggtcgattcatgggaaaggggagtggatgaccacggaagacatgcttgaggtgtggaacagagtatggataaccaacaacccacacatgcaggacaagacaatggtgaaaaaatggagagatgtcccttatctaaccaagagacaagacaagctgtgcggatcactgattggaatgaccaatagggccacctgggcctcccacatccatttagtcatccatcgtatccgaacgctgattggacaggagaaatacactgactacctaacagtcatggacaggtattctgtggatgctgacctgcaactgggtgagcttatctgaaacaccatctaacaggaataaccgggatacaaaccacgggtggagaaccggactccccacaacctgaaaccgggatataaaccacggctggagaaccgggctccgcacttaaaatgaaacagaaaccgggataaaaactacggatggagaaccggactccacacattgagacagaagaagttgtcagcccagaaccccacacgagttttgccactgctaagctgtgaggcagtgcaggctgggacagccgacctccaggttgcgaaaaacctggtttctgggacctcccaccccagagtaaaaagaacggagcctccgctaccaccctcccacgtggtggtagaaagacggggtctagaggttagaggagaccctccagggaacaaatagtgggaccatattgacgccagggaaagaccggagtggttctctgcttttcctccagaggtctgtgagcacagtttgctcaagaataagcagacctttggatgacaaacacaaaaccac

SEQ ID NO: 10 - protein, 3767 aa, Yellow fever virus
MSGRKAQGKTLGVNMVRRGVRSLSNKIKQKTKQIGNRPGPSRGVQGFIFFFLFNILTGKKITAHLKRLWKMLDPRQGLAVLRKVKRVVASLMRGLSSRKRRSHDVLTVQFLILGMLLMTGGVTLVRKNRWLLLNVTSEDLGKTFSVGTGNCTTNILEAKYWCPDSMEYNCPNLSPREEPDDIDCWCYGVENVRVAYGKCDSAGRSRRSRRAIDLPTHENHGLKTRQEKWMTGRMGERQLQKIERWFVRNPFFAVTALTIAYLVGSNMTQRVVIALLVLAVGPAYSAHCIGITDRDFIEGVHGGTWVSATLEQDKCVTVMAPDKPSLDISLETVAIDRPAEARKVCYNAVLTHVKINDKCPSTGEAHLAEENEGDNACKRTYSDRGWGNGCGLFGKGSIVACAKFTCAKSMSLFEVDQTKIQYVIRAQLHVGAKQENWNTSIKTLKFDALSGSQEVEFIGYGKATLECQVQTAVDFGNSYIAEMETESWIVDRQWAQDLTLPWQSGSGGVWREMHHLVEFEPPHAATIRVLALGNQEGSLKTALTGAMRVTKDTNDNNLYKLHGGHVSCRVKLSALTLKGTSYKICTDKMFFVKNPTDTGHGTVVMQVKVSKGAPCRIPVIVADDLTAAINKGILVTVNPIASTNDDEVLIEVNPPFGDSYIIVGRGDSRLTYQWHKEGSSIGKLFTQTMKGVERLAVMGDTAWDFSSAGGFFTSVGKGIHTVFGSAFQGLFGGLNWITKVIMGAVLIWVGINTRNMTMSMSMILVGVIMMFLSLGVGADQGCAINFGRKSGEEHAVGNTTGSSKGEELFTGVVPILVELDGDVNGHKFSVSGEGEGDATYGKLTLKFICTTGKLPVPWPTLVTTLTYGVQCFSRYPDHMKQHDFFKSAMPEGYVQERTIFFKDDGNYKTRAEVKFEGDTLVNRIELKGIDFKEDGNILGHKLEYNYNSHNVYIMADKQKNGIKVNFKIRHNIEDGSVQLADHYQQNTPIGDGPVLLPDNHYLSTQSALSKDPNEKRDHMVLLEFVTAAGITLGMDELYKSGGKQEGSRTRRSVLIPSHAQGKEGSSIGTSLGKAVHQVFGSVYTTMFGGVSWMIRILIGFLVLWIGTNSRNTSMAMTCIAVGGITLFLGFTVGADQGCAINFGKRELKCGDGIFIFRDSDDWLNKYSYYPEDPVKLASIVKASFEEGKCGLNSVDSLEHEMWRSRADEINAIFEENEVDISVVVQDPKNVYQRGTHPFSRIRDGLQYGWKTWGKNLVFSPGRKNGSFIIDGKSRKECPFSNRVWNSFQIEEFGTGVFTTRVYMDAVFEYTIDCDGSILGAAVNGKKSAHGSPTFWMGSHEVNGTWMIHTLEALDYKECEWPLTHTIGTSVEESEMFMPRSIGGPVSSHNHIPGYKVQTNGPWMQVPLEVKREACPGTSVIIDGNCDGRGKSTRSTTDSGKVIPEWCCRSCTMPPVSFHGSDGCWYPMEIRPRKTHESHLVRSWVTAGEIHAVPFGLVSMMIAMEVVLRKRQGPKQMLVGGVVLLGAMLVGQVTLLDLLKLTVAVGLHFHEMNNGGDAMYMALIAAFSIRPGLLIGFGLRTLWSPRERLVLTLGAAMVEIALGGVMGGLWKYLNAVSLCILTINAVASRKASNTILPLMALLTPVTMAEVRLAAMFFCAMVIIGVLHQNFKDTSMQKTIPLVALTLTSYLGLTQPFLGLCAFLATRIFGRRSIPVNEALAAAGLVGVLAGLAFQEMENFLGPIAVGGLLMMLVSVAGRVDGLELKKLGEVSWEEEAEISGSSARYDVALSEQGEFKLLSEEKVPWDQVVMTSLALVGAALHPFALLLVLAGWLFHVRGARRSGDVLWDIPTPKIIEECEHLEDGIYGIFQSTFLGASQRGVGVAQGGVFHTMWHVTRGAFLVRNGKKLIPSWASVKEDLVAYGGSWKLEGRWDGEEEVQLIAAVPGKNVVNVQTKPSLFKVRNGGEIGAVALDYPSGTSGSPIVNRNGEVIGLYGNGILVGDNSFVSAISQTEVKEEGKEELQEIPTMLKKGMTTVLDFHPGAGKTRRFLPQILAECARRRLRTLVLAPTRVVLSEMKEAFHGLDVKFHTQAFSAHGSGREVIDAMCHATLTYRMLEPTRVVNWEVIIMDEAHFLDPASIAARGWAAHRARANESATILMTATPPGTSDEFPHSNGEIEDVQTDIPSEPWNTGHDWILADKRPTAWFLPSIRAANVMAASLRKAGKSVVVLNRKTFEREYPTIKQKKPDFILATDIAEMGANLCVERVLDCRTAFKPVLVDEGRKVAIKGPLRISASSAAQRRGRIGRNPNRDGDSYYYSEPTSENNAHHVCWLEASMLLDNMEVRGGMVAPLYGVEGTKTPVSPGEMRLRDDQRKVFRELVRNCDLPVWLSWQVAKAGLKTNDRKWCFEGPEEHEILNDSGETVKCRAPGGAKKPLRPRWCDERVSSDQSALSEFIKFAEGRRGAAEVLVVLSELPDFLAKKGGEAMDTISVFLHSEEGSRAYRNALSMMPEAMTIVMLFILAGLLTSGMVIFFMSPKGISRMSMAMGTMAGCGYLMFLGGVKPTHISYVMLIFFVLMVVVIPEPGQQRSIQDNQVAYLIIGILTLVSAVAANELGMLEKTKEDLFGKKNLIPSSASPWSWPDLDLKPGAAWTVYVGIVTMLSPMLHHWIKVEYGNLSLSGIAQSASVLSFMDKGIPFMKMNISVIMLLVSGWNSITVMPLLCGIGCAMLHWSLILPGIKAQQSKLAQRRVFHGVAKNPVVDGNPTVDIEEAPEMPALYEKKLALYLLLALSLASVAMCRTPFSLAEGIVLASAALGPLIEGNTSLLWNGPMAVSMTGVMRGNHYAFVGVMYNLWKMKTGRRGSANGKTLGEVWKRELNLLDKRQFELYKRTDIVEVDRDTARRHLAEGKVDTGVAVSRGTAKLRWFHERGYVKLEGRVIDLGCGRGGWCYYAAAQKEVSGVKGFTLGRDGHEKPMNVQSLGWNIITFKDKTDIHRLEPVKCDTLLCDIGESSSSSVTEGERTVRVLDTVEKWLACGVDNFCVKVLAPYMPDVLEKLELLQRRFGGTVIRNPLSRNSTHEMYYVSGARSNVTFTVNQTSRLLMRRMRRPTGKVTLEADVILPIGTRSVETDKGPLDKEAIEERVERIKSEYMTSWFYDNDNPYRTWHYCGSYVTKTSGSAASMVNGVIKILTYPWDRIEEVTRMAMTDTTPFGQQRVFKEKVDTRAKDPPAGTRKIMKVVNRWLFRHLAREKSPRLCTKEEFIAKVRSHAAIGAYLEEQEQWKTANEAVQDPKFWELVDEERKLHQQGRCRTCVYNMMGKREKKLSEFGKAKGSRAIWYMWLGARYLEFEALGFLNEDHWASRENSGGGVEGIGLQYLGYVIRDLAAMDGGGFYADDTAGWDTRITEADLDDEQEILNYMSPHHKKLAQAVMEMTYKNKVVKVLRPAPGGKAYMDVISRRDQRGSGQVVTYALNTITNLKVQLIRMAEAEMVIHHQHVQDCDESVLTRLEAWLTEHGCNRLKRMAVSGDDCVVRPIDDRFGLALSHLNAMSKVRKDISEWQPSKGWNDWENVPFCSHHFHELQLKDGRRIVVPCREQDELIGRGRVSPGNGWMIKETACLSKAYANMWSLMYFHKRDMRLLSLAVSSAVPTSWVPQGRTTWSIHGKGEWMTTEDMLEVWNRVWITNNPHMQDKTMVKKWRDVPYLTKRQDKLCGSLIGMTNRATWASHIHLVIHRIRTLIGQEKYTDYLTVMDRYSVDADLQLGELI

SEQ ID NO: 11 - DNA, 12046 bp, Yellow fever virus
agtaaatcctgtgtgctaattgaggtgcattggtctgcaaatcgagttgctaggcaataaacacatttggattaattttaatcgttcgttgagcgattagcagagaactgaccagaacatgtctggtcgtaaagctcagggaaaaaccctgggcgtcaatatggtacgacgaggagttcgctccttgtcaaacaaaataaaacaaaaaacaaaacaaattggaaacagacctggaccttcaagaggtgttcaaggatttatctttttctttttgttcaacattttgactggaaaaaagatcacagcccacctaaagaggttgtggaaaatgctggacccaagacaaggcttggctgttctaaggaaagtcaagagagtggtggccagtttgatgagaggattgtcctcaaggaaacgccgttcccatgatgttctgactgtgcaattcctaattttgggaatgctgttgatgaccggtggagtgaccttggtgcggaaaaacagatggttgctcctaaatgtgacatctgaggacctcgggaaaacattctctgtgggcacaggcaactgcacaacaaacattttggaagccaagtactggtgcccagactcaatggaatacaactgtcccaatctcagtccaagagaggagccagatgacattgattgctggtgctatggggtggaaaacgttagagtcgcatatggtaagtgtgactcagcaggcaggtctaggaggtcaagaagggccattgacttgcctacgcatgaaaaccatggtttgaagacccggcaagaaaaatggatgactggaagaatgggtgaaaggcaactccaaaagattgagagatggttcgtgaggaaccccttttttgcagtgacggctctgaccattgcctaccttgtgggaagcaacatgacgcaacgagtcgtgattgccctactggtcttggctgttggtccggcctactcagctcactgcattggaattactgacagggatttcattgagggggtgcatggaggaacttgggtttcagctaccctggagcaagacaagtgtgtcactgttatggcccctgacaagccttcattggacatctcactagagacagtagccattgatagacctgctgaggcgaggaaagtgtgttacaatgcagttctcactcatgtgaagattaatgacaagtgccccagcactggagaggcccacctagctgaagagaacgaaggggacaatgcgtgcaagcgcacttattctgatagaggctggggcaatggctgtggcctatttgggaaagggagcattgtggcatgcgccaaattcacttgtgccaaatccatgagtttgtttgaggttgatcagaccaaaattcagtatgtcatcagagcacaattgcatgtaggggccaagcaggaaaattggaataccagcattaagactctcaagtttgatgccctgtcaggctcccaggaagtcgagttcattgggtatggaaaagctacactggaatgccaggtgcaaactgcggtggactttggtaacagttacatcgctgagatggaaacagagagctggatagtggacagacagtgggcccaggacttgaccctgccatggcagagtggaagtggcggggtgtggagagagatgcatcatcttgtcgaatttgaacctccgcatgccgccactatcagagtactggccctgggaaaccaggaaggctccttgaaaacagctcttactggcgcaatgagggttacaaaggacacaaatgacaacaacctttacaaactacatggtggacatgtttcttgcagagtgaaattgtcagctttgacactcaaggggacatcctacaaaatatgcactgacaaaatgttttttgtcaagaacccaactgacactggccatggcactgttgtgatgcaggtgaaagtgtcaaaaggagccccctgcaggattccagtgatagtagctgatgatcttacagcggcaatcaataaaggcattttggttacagttaaccccatcgcctcaaccaatgatgatgaagtgctgattgaggtgaacccaccttttggagacagctacattatcgttgggagaggagattcacgtctcacttaccagtggcacaaagagggaagctcaataggaaagttgttcactcagaccatgaaaggcgtggaacgcctggccgtcatgggagacaccgcctgggatttcagctccgctggagggttcttcacttcggttgggaaaggaattcatacggtgtttggctctgcctttcaggggctatttggcggcttgaactggataacaaaggtcatcatgggggcggtacttatatgggttggcatcaacacaagaaacatgacaatgtccatgagcatgatcttggtaggagtgatcatgatgtttttgtctctaggagttggggcggatcaaggatgcgccatcaacttcggccgaaagggatcacaaacctccaacacaactaaatgggctcctcccggacaaggaagtcccgggagcaagggcgaggagctgttcaccggggtggtgcccatcctggtcgagctggacggcgacgtaaacggccacaagttcagcgtgtccggcgagggcgagggcgatgccacctacggcaagctgaccctgaagttcatctgcaccaccggcaagctgcccgtgccctggcccaccctcgtgaccaccctgacctacggcgtgcagtgcttcagccgctaccccgaccacatgaagcagcacgacttcttcaagtccgccatgcccgaaggctacgtccaggagcgcaccatcttcttcaaggacgacggcaactacaagacccgcgccgaggtgaagttcgagggcgacaccctggtgaaccgcatcgagctgaagggcatcgacttcaaggaggacggcaacatcctggggcacaagctggagtacaactacaacagccacaacgtctatatcatggccgacaagcagaagaacggcatcaaggtgaacttcaagatccgccacaacatcgaggacggcagcgtgcagctcgccgaccactaccagcagaacacccccatcggcgacggccccgtgctgctgcccgacaaccactacctgagcacccagtccgccctgagcaaagaccccaacgagaagcgcgatcacatggtcctgctggagttcgtgaccgccgccgggatcactctcggcatggacgagctgtacaagtccggaagcagtccacagctgttgaattttgaccttcttaagcttgctggagacgtcgagtccaaccctgggccaaaggagggaagctcaataggaaagatgtttgagtccacatacagaggtgcaaaacgaatggccattctaggtgaaacagcttgggattttggttccgttggtggactgttcacatcattgggaaaggctgtgcaccaggtttttggaagtgtgtatacaaccatgtttggaggagtctcatggatgattagaatcctaattgggttcttagtgttgtggattggcacgaactccaggaacacttcaatggctatgacgtgcatagctgttggaggaatcactctgtttctgggcttcacagttggcgccgatcaaggatgcgccatcaactttggcaagagagagctcaagtgcggagatggtatcttcatatttagagactctgatgactggctgaacaagtactcatactatccagaagatcctgtgaagcttgcatcaatagtgaaagcctcttttgaagaagggaagtgtggcctaaattcagttgactcccttgagcatgagatgtggagaagcagggcagatgagatcaatgccatttttgaggaaaacgaggtggacatttctgttgtcgtgcaggatccaaagaatgtttaccagagaggaactcatccattttccagaattcgggatggtctgcagtatggttggaagacttggggtaagaaccttgtgttctccccagggaggaagaatggaagcttcatcatagatggaaagtccaggaaagaatgcccgttttcaaaccgggtctggaattctttccagatagaggagtttgggacgggagtgttcaccacacgcgtgtacatggacgcagtctttgaatacaccatagactgcgatggatctatcttgggtgcagcggtgaacggaaaaaagagtgcccatggctctccaacattttggatgggaagtcatgaagtaaatgggacatggatgatccacaccttggaggcattagattacaaggagtgtgagtggccactgacacatacgattggaacatcagttgaagagagtgaaatgttcatgccgagatcaatcggaggcccagttagctctcacaatcatatccctggatacaaggttcagacgaacggaccttggatgcaggtaccactagaagtgaagagagaagcttgcccagggactagcgtgatcattgatggcaactgtgatggacggggaaaatcaaccagatccaccacggatagcgggaaagttattcctgaatggtgttgccgctcctgcacaatgccgcctgtgagcttccatggtagtgatgggtgttggtatcccatggaaattaggccaaggaaaacgcatgaaagccatctggtgcgctcctgggttacagctggagaaatacatgctgtcccttttggtttggtgagcatgatgatagcaatggaagtggtcctaaggaaaagacagggaccaaagcaaatgttggttggaggagtagtgctcttgggagcaatgctggtcgggcaagtaactctccttgatttgctgaaactcacagtggctgtgggattgcatttccatgagatgaacaatggaggagacgccatgtatatggcgttgattgctgccttttcaatcagaccagggctgctcatcggctttgggctcaggaccctatggagccctcgggaacgccttgtgctgaccctaggagcagccatggtggagattgccttgggtggcgtgatgggcggcctgtggaagtatctaaatgcagtttctctctgcatcctgacaataaatgctgttgcttctaggaaagcatcaaataccatcttgcccctcatggctctgttgacacctgtcactatggctgaggtgagacttgccgcaatgttcttttgtgccatggttatcataggggtccttcaccagaatttcaaggacacctccatgcagaagactatacctctggtggccctcacactcacatcttacctgggcttgacacaaccttttttgggcctgtgtgcatttctggcaacccgcatatttgggcgaaggagtatcccagtgaatgaggcactcgcagcagctggtctagtgggagtgctggcaggactggcttttcaggagatggagaacttccttggtccgattgcagttggaggactcctgatgatgctggttagcgtggctgggagggtggatgggctagagctcaagaagcttggtgaagtttcatgggaagaggaggcggagatcagcgggagttccgcccgctatgatgtggcactcagtgaacaaggggagttcaagctgctttctgaagagaaagtgccatgggaccaggttgtgatgacctcgctggccttggttggggctgccctccatccatttgctcttctgctggtccttgctgggtggctgtttcatgtcaggggagctaggagaagtggggatgtcttgtgggatattcccactcctaagatcatcgaggaatgtgaacatctggaggatgggatttatggcatattccagtcaaccttcttgggggcctcccagcgaggagtgggagtggcacagggaggggtgttccacacaatgtggcatgtcacaagaggagctttccttgtcaggaatggcaagaagttgattccatcttgggcttcagtaaaggaagaccttgtcgcctatggtggctcatggaagttggaaggcagatgggatggagaggaagaggtccagttgatcgcggctgttccaggaaagaacgtggtcaacgtccagacaaaaccgagcttgttcaaagtgaggaatgggggagaaatcggggctgtcgctcttgactatccgagtggcacttcaggatctcctattgttaacaggaacggagaggtgattgggctgtacggcaatggcatccttgtcggtgacaactccttcgtgtccgccatatcccagactgaggtgaaggaagaaggaaaggaggagctccaagagatcccgacaatgctaaagaaaggaatgacaactgtccttgattttcatcctggagctgggaagacaagacgtttcctcccacagatcttggccgagtgcgcacggagacgcttgcgcactcttgtgttggcccccaccagggttgttctttctgaaatgaaggaggcttttcacggcctggacgtgaaattccacacacaggctttttccgctcacggcagcgggagagaagtcattgatgccatgtgccatgccaccctaacttacaggatgttggaaccaactagggttgttaactgggaagtgatcattatggatgaagcccattttttggatccagctagcatagccgctagaggttgggcagcgcacagagctagggcaaatgaaagtgcaacaatcttgatgacagccacaccgcctgggactagtgatgaatttccacattcaaatggtgaaatagaagatgttcaaacggacatacccagtgagccctggaacacagggcatgactggatcctggctgacaaaaggcccacggcatggttccttccatccatcagagctgcaaatgtcatggctgcctctttgcgtaaggctggaaagagtgtggtggtcctgaacaggaaaacctttgagagagaataccccacgataaagcagaagaaacctgactttatattggccactgacatagctgaaatgggagccaacctttgcgtggagcgagtgctggattgcaggacggcttttaagcctgtgcttgtggatgaagggaggaaggtggcaataaaagggccacttcgtatctccgcatcctctgctgctcaaaggagggggcgcattgggagaaatcccaacagagatggagactcatactactattctgagcctacaagtgaaaataatgcccaccacgtctgctggttggaggcctcaatgctcttggacaacatggaggtgaggggtggaatggtcgccccactctatggcgttgaaggaactaaaacaccagtttcccctggtgaaatgagactgagggatgaccagaggaaagtcttcagagaactagtgaggaattgtgacctgcccgtttggctttcgtggcaagtggccaaggctggtttgaagacgaatgatcgtaagtggtgttttgaaggccctgaggaacatgagatcttgaatgacagcggtgaaacagtgaagtgcagggctcctggaggagcaaagaagcctctgcgcccaaggtggtgtgatgaaagggtgtcatctgaccagagtgcgctgtctgaatttattaagtttgctgaaggtaggaggggagctgctgaagtgctagttgtgctgagtgaactccctgatttcctggctaaaaaaggtggagaggcaatggataccatcagtgtgttcctccactctgaggaaggctctagggcttaccgcaatgcactatcaatgatgcctgaggcaatgacaatagtcatgctgtttatactggctggactactgacatcgggaatggtcatctttttcatgtctcccaaaggcatcagtagaatgtctatggcgatgggcacaatggccggctgtggatatctcatgttccttggaggcgtcaaacccactcacatctcctatgtcatgctcatattctttgtcctgatggtggttgtgatccccgagccagggcaacaaaggtccatccaagacaaccaagtggcatacctcattattggcatcctgacgctggtttcagcggtggcagccaacgagctaggcatgctggagaaaaccaaagaggacctctttgggaagaagaacttaattccatctagtgcttcaccctggagttggccggatcttgacctgaagccaggagctgcctggacagtgtacgttggcattgttacaatgctctctccaatgttgcaccactggatcaaagtcgaatatggcaacctgtctctgtctggaatagcccagtcagcctcagtcctttctttcatggacaaggggataccattcatgaagatgaatatctcggtcataatgctgctggtcagtggctggaattcaataacagtgatgcctctgctctgtggcatagggtgcgccatgctccactggtctctcattttacctggaatcaaagcgcagcagtcaaagcttgcacagagaagggtgttccatggcgttgccaagaaccctgtggttgatgggaatccaacagttgacattgaggaagctcctgaaatgcctgccctttatgagaagaaactggctctatatctccttcttgctctcagcctagcttctgttgccatgtgcagaacgcccttttcattggctgaaggcattgtcctagcatcagctgccttagggccgctcatagagggaaacaccagccttctttggaatggacccatggctgtctccatgacaggagtcatgagggggaatcactatgcttttgtgggagtcatgtacaatctatggaagatgaaaactggacgccgggggagcgcgaatggaaaaactttgggtgaagtctggaagagggaactgaatctgttggacaagcgacagtttgagttgtataaaaggaccgacattgtggaggtggatcgtgatacggcacgcaggcatttggccgaagggaaggtggacaccggggtggcggtctccagggggaccgcaaagttaaggtggttccatgagcgtggctatgtcaagctggaaggtagggtgattgacctggggtgtggccgcggaggctggtgttactacgctgctgcgcaaaaggaagtgagtggggtcaaaggatttactcttggaagagacggccatgagaaacccatgaatgtgcaaagtctgggatggaacatcatcaccttcaaggacaaaactgatatccaccgcctagaaccagtgaaatgtgacacccttttgtgtgacattggagagtcatcatcgtcatcggtcacagagggggaaaggaccgtgagagttcttgatactgtagaaaaatggctggcttgtggggttgacaacttctgtgtgaaggtgttagctccatacatgccagatgttcttgagaaactggaattgctccaaaggaggtttggcggaacagtgatcaggaaccctctctccaggaattccactcatgaaatgtactacgtgtctggagcccgcagcaatgtcacatttactgtgaaccaaacatcccgcctcctgatgaggagaatgaggcgtccaactggaaaagtgaccctggaggctgacgtcatcctcccaattgggacacgcagtgttgagacagacaagggacccctggacaaagaggccatagaagaaagggttgagaggataaaatctgagtacatgacctcttggttttatgacaatgacaacccctacaggacctggcactactgtggctcctatgtcacaaaaacctcaggaagtgcggcgagcatggtaaatggtgttattaaaattctgacatatccatgggacaggatagaggaggtcaccagaatggcaatgactgacacaaccccttttggacagcaaagagtgtttaaagaaaaagttgacaccagagcaaaggatccaccagcgggaactaggaagatcatgaaagttgtcaacaggtggctgttccgccacctggccagagaaaagagccccagactgtgcacaaaggaagaatttattgcaaaagtccgaagtcatgcagccattggagcttacctggaagaacaagaacagtggaagactgccaatgaggctgtccaagacccaaagttctgggaactggtggatgaagaaaggaagctgcaccaacaaggcaggtgtcggacttgtgtgtacaacatgatggggaaaagagagaagaagctgtcagagtttgggaaagcaaagggaagccgtgccatatggtatatgtggctgggagcgcggtatcttgagtttgaggccctgggattcctgaatgaggaccattgggcttccagggaaaactcaggaggaggagtggaaggcattggcttacaatacctaggatatgtgatcagagacctggctgcaatggatggtggtggattctacgcggatgacaccgctggatgggacacgcgcatcacagaggcagaccttgatgatgaacaggagatcttgaactacatgagcccacatcacaaaaaactggcacaagcagtgatggaaatgacatacaagaacaaagtggtgaaagtgttgagaccagccccaggagggaaagcctacatggatgtcataagtcgacgagaccagagaggatccgggcaggtagtgacttatgctctgaacaccatcaccaacttgaaagtccaattgatcagaatggcagaagcagagatggtgatacatcaccaacatgttcaagattgtgatgaatcagttctgaccaggctggaggcatggctcactgagcacggatgtaacagactgaagaggatggcggtgagtggagacgactgtgtggtccggcccatcgatgacaggttcggcctggccctgtcccatctcaacgccatgtccaaggttagaaaggacatatctgaatggcagccatcaaaagggtggaatgattgggagaatgtgcccttctgttcccaccacttccatgaactacagctgaaggatggcaggaggattgtggtgccttgccgagaacaggacgagctcattgggagaggaagggtgtctccaggaaacggctggatgatcaaggaaacagcttgcctcagcaaagcctatgccaacatgtggtcactgatgtattttcacaaaagggacatgaggctactgtcattggctgtttcctcagctgttcccacctcatgggttccacaaggacgcacaacatggtcgattcatgggaaaggggagtggatgaccacggaagacatgcttgaggtgtggaacagagtatggataaccaacaacccacacatgcaggacaagacaatggtgaaaaaatggagagatgtcccttatctaaccaagagacaagacaagctgtgcggatcactgattggaatgaccaatagggccacctgggcctcccacatccatttagtcatccatcgtatccgaacgctgattggacaggagaaatacactgactacctaacagtcatggacaggtattctgtggatgctgacctgcaactgggtgagcttatctgaaacaccatctaacaggaataaccgggatacaaaccacgggtggagaaccggactccccacaacctgaaaccgggatataaaccacggctggagaaccgggctccgcacttaaaatgaaacagaaaccgggataaaaactacggatggagaaccggactccacacattgagacagaagaagttgtcagcccagaaccccacacgagttttgccactgctaagctgtgaggcagtgcaggctgggacagccgacctccaggttgcgaaaaacctggtttctgggacctcccaccccagagtaaaaagaacggagcctccgctaccaccctcccacgtggtggtagaaagacggggtctagaggttagaggagaccctccagggaacaaatagtgggaccatattgacgccagggaaagaccggagtggttctctgcttttcctccagaggtctgtgagcacagtttgctcaagaataagcagacctttggatgacaaacacaaaaccac

SEQ ID NO: 12 - protein, 3806 aa, Yellow fever virus
MSGRKAQGKTLGVNMVRRGVRSLSNKIKQKTKQIGNRPGPSRGVQGFIFFFLFNILTGKKITAHLKRLWKMLDPRQGLAVLRKVKRVVASLMRGLSSRKRRSHDVLTVQFLILGMLLMTGGVTLVRKNRWLLLNVTSEDLGKTFSVGTGNCTTNILEAKYWCPDSMEYNCPNLSPREEPDDIDCWCYGVENVRVAYGKCDSAGRSRRSRRAIDLPTHENHGLKTRQEKWMTGRMGERQLQKIERWFVRNPFFAVTALTIAYLVGSNMTQRVVIALLVLAVGPAYSAHCIGITDRDFIEGVHGGTWVSATLEQDKCVTVMAPDKPSLDISLETVAIDRPAEARKVCYNAVLTHVKINDKCPSTGEAHLAEENEGDNACKRTYSDRGWGNGCGLFGKGSIVACAKFTCAKSMSLFEVDQTKIQYVIRAQLHVGAKQENWNTSIKTLKFDALSGSQEVEFIGYGKATLECQVQTAVDFGNSYIAEMETESWIVDRQWAQDLTLPWQSGSGGVWREMHHLVEFEPPHAATIRVLALGNQEGSLKTALTGAMRVTKDTNDNNLYKLHGGHVSCRVKLSALTLKGTSYKICTDKMFFVKNPTDTGHGTVVMQVKVSKGAPCRIPVIVADDLTAAINKGILVTVNPIASTNDDEVLIEVNPPFGDSYIIVGRGDSRLTYQWHKEGSSIGKLFTQTMKGVERLAVMGDTAWDFSSAGGFFTSVGKGIHTVFGSAFQGLFGGLNWITKVIMGAVLIWVGINTRNMTMSMSMILVGVIMMFLSLGVGADQGCAINFGRKGSQTSNTTKWAPPGQGSPGSKGEELFTGVVPILVELDGDVNGHKFSVSGEGEGDATYGKLTLKFICTTGKLPVPWPTLVTTLTYGVQCFSRYPDHMKQHDFFKSAMPEGYVQERTIFFKDDGNYKTRAEVKFEGDTLVNRIELKGIDFKEDGNILGHKLEYNYNSHNVYIMADKQKNGIKVNFKIRHNIEDGSVQLADHYQQNTPIGDGPVLLPDNHYLSTQSALSKDPNEKRDHMVLLEFVTAAGITLGMDELYKSGSSPQLLNFDLLKLAGDVESNPGPKEGSSIGKMFESTYRGAKRMAILGETAWDFGSVGGLFTSLGKAVHQVFGSVYTTMFGGVSWMIRILIGFLVLWIGTNSRNTSMAMTCIAVGGITLFLGFTVGADQGCAINFGKRELKCGDGIFIFRDSDDWLNKYSYYPEDPVKLASIVKASFEEGKCGLNSVDSLEHEMWRSRADEINAIFEENEVDISVVVQDPKNVYQRGTHPFSRIRDGLQYGWKTWGKNLVFSPGRKNGSFIIDGKSRKECPFSNRVWNSFQIEEFGTGVFTTRVYMDAVFEYTIDCDGSILGAAVNGKKSAHGSPTFWMGSHEVNGTWMIHTLEALDYKECEWPLTHTIGTSVEESEMFMPRSIGGPVSSHNHIPGYKVQTNGPWMQVPLEVKREACPGTSVIIDGNCDGRGKSTRSTTDSGKVIPEWCCRSCTMPPVSFHGSDGCWYPMEIRPRKTHESHLVRSWVTAGEIHAVPFGLVSMMIAMEVVLRKRQGPKQMLVGGVVLLGAMLVGQVTLLDLLKLTVAVGLHFHEMNNGGDAMYMALIAAFSIRPGLLIGFGLRTLWSPRERLVLTLGAAMVEIALGGVMGGLWKYLNAVSLCILTINAVASRKASNTILPLMALLTPVTMAEVRLAAMFFCAMVIIGVLHQNFKDTSMQKTIPLVALTLTSYLGLTQPFLGLCAFLATRIFGRRSIPVNEALAAAGLVGVLAGLAFQEMENFLGPIAVGGLLMMLVSVAGRVDGLELKKLGEVSWEEEAEISGSSARYDVALSEQGEFKLLSEEKVPWDQVVMTSLALVGAALHPFALLLVLAGWLFHVRGARRSGDVLWDIPTPKIIEECEHLEDGIYGIFQSTFLGASQRGVGVAQGGVFHTMWHVTRGAFLVRNGKKLIPSWASVKEDLVAYGGSWKLEGRWDGEEEVQLIAAVPGKNVVNVQTKPSLFKVRNGGEIGAVALDYPSGTSGSPIVNRNGEVIGLYGNGILVGDNSFVSAISQTEVKEEGKEELQEIPTMLKKGMTTVLDFHPGAGKTRRFLPQILAECARRRLRTLVLAPTRVVLSEMKEAFHGLDVKFHTQAFSAHGSGREVIDAMCHATLTYRMLEPTRVVNWEVIIMDEAHFLDPASIAARGWAAHRARANESATILMTATPPGTSDEFPHSNGEIEDVQTDIPSEPWNTGHDWILADKRPTAWFLPSIRAANVMAASLRKAGKSVVVLNRKTFEREYPTIKQKKPDFILATDIAEMGANLCVERVLDCRTAFKPVLVDEGRKVAIKGPLRISASSAAQRRGRIGRNPNRDGDSYYYSEPTSENNAHHVCWLEASMLLDNMEVRGGMVAPLYGVEGTKTPVSPGEMRLRDDQRKVFRELVRNCDLPVWLSWQVAKAGLKTNDRKWCFEGPEEHEILNDSGETVKCRAPGGAKKPLRPRWCDERVSSDQSALSEFIKFAEGRRGAAEVLVVLSELPDFLAKKGGEAMDTISVFLHSEEGSRAYRNALSMMPEAMTIVMLFILAGLLTSGMVIFFMSPKGISRMSMAMGTMAGCGYLMFLGGVKPTHISYVMLIFFVLMVVVIPEPGQQRSIQDNQVAYLIIGILTLVSAVAANELGMLEKTKEDLFGKKNLIPSSASPWSWPDLDLKPGAAWTVYVGIVTMLSPMLHHWIKVEYGNLSLSGIAQSASVLSFMDKGIPFMKMNISVIMLLVSGWNSITVMPLLCGIGCAMLHWSLILPGIKAQQSKLAQRRVFHGVAKNPVVDGNPTVDIEEAPEMPALYEKKLALYLLLALSLASVAMCRTPFSLAEGIVLASAALGPLIEGNTSLLWNGPMAVSMTGVMRGNHYAFVGVMYNLWKMKTGRRGSANGKTLGEVWKRELNLLDKRQFELYKRTDIVEVDRDTARRHLAEGKVDTGVAVSRGTAKLRWFHERGYVKLEGRVIDLGCGRGGWCYYAAAQKEVSGVKGFTLGRDGHEKPMNVQSLGWNIITFKDKTDIHRLEPVKCDTLLCDIGESSSSSVTEGERTVRVLDTVEKWLACGVDNFCVKVLAPYMPDVLEKLELLQRRFGGTVIRNPLSRNSTHEMYYVSGARSNVTFTVNQTSRLLMRRMRRPTGKVTLEADVILPIGTRSVETDKGPLDKEAIEERVERIKSEYMTSWFYDNDNPYRTWHYCGSYVTKTSGSAASMVNGVIKILTYPWDRIEEVTRMAMTDTTPFGQQRVFKEKVDTRAKDPPAGTRKIMKVVNRWLFRHLAREKSPRLCTKEEFIAKVRSHAAIGAYLEEQEQWKTANEAVQDPKFWELVDEERKLHQQGRCRTCVYNMMGKREKKLSEFGKAKGSRAIWYMWLGARYLEFEALGFLNEDHWASRENSGGGVEGIGLQYLGYVIRDLAAMDGGGFYADDTAGWDTRITEADLDDEQEILNYMSPHHKKLAQAVMEMTYKNKVVKVLRPAPGGKAYMDVISRRDQRGSGQVVTYALNTITNLKVQLIRMAEAEMVIHHQHVQDCDESVLTRLEAWLTEHGCNRLKRMAVSGDDCVVRPIDDRFGLALSHLNAMSKVRKDISEWQPSKGWNDWENVPFCSHHFHELQLKDGRRIVVPCREQDELIGRGRVSPGNGWMIKETACLSKAYANMWSLMYFHKRDMRLLSLAVSSAVPTSWVPQGRTTWSIHGKGEWMTTEDMLEVWNRVWITNNPHMQDKTMVKKWRDVPYLTKRQDKLCGSLIGMTNRATWASHIHLVIHRIRTLIGQEKYTDYLTVMDRYSVDADLQLGELI

SEQ ID NO: 13 - DNA, 939 bp, Yellow fever virus
gatcaaggatgcgccatcaactttggcgtgagcaagggcgaggagctgttcaccggggtggtgcccatcctggtcgagctggacggcgacgtaaacggccacaagttcagcgtgtccggcgagggcgagggcgatgccacctacggcaagctgaccctgaagttcatctgcaccaccggcaagctgcccgtgccctggcccaccctcgtgaccaccctgacctacggcgtgcagtgcttcagccgctaccccgaccacatgaagcagcacgacttcttcaagtccgccatgcccgaaggctacgtccaggagcgcaccatcttcttcaaggacgacggcaactacaagacccgcgccgaggtgaagttcgagggcgacaccctggtgaaccgcatcgagctgaagggcatcgacttcaaggaggacggcaacatcctggggcacaagctggagtacaactacaacagccacaacgtctatatcatggccgacaagcagaagaacggcatcaaggtgaacttcaagatccgccacaacatcgaggacggcagcgtgcagctcgccgaccactaccagcagaacacccccatcggcgacggccccgtgctgctgcccgacaaccactacctgagcacccagtccgccctgagcaaagaccccaacgagaagcgcgatcacatggtcctgctggagttcgtgaccgccgccgggatcactctcggcatggacgagctgtacaagacatcattgggaaaggctgtgcaccaggtttttggaagtgtgtatacaaccatgtttggaggagtctcatggatgattagaatcctaattgggttcttagtgttgtggattggcacgaactcgaggaacacttcaatggctatgacgtgcatagctgttggaggaatcactctgtttctgggcttcacagttggcgcc

SEQ ID NO: 14 - protein, 313 aa, Yellow fever virus
DQGCAINFGVSKGEELFTGVVPILVELDGDVNGHKFSVSGEGEGDATYGKLTLKFICTTGKLPVPWPTLVTTLTYGVQCFSRYPDHMKQHDFFKSAMPEGYVQERTIFFKDDGNYKTRAEVKFEGDTLVNRIELKGIDFKEDGNILGHKLEYNYNSHNVYIMADKQKNGIKVNFKIRHNIEDGSVQLADHYQQNTPIGDGPVLLPDNHYLSTQSALSKDPNEKRDHMVLLEFVTAAGITLGMDELYKTSLGKAVHQVFGSVYTTMFGGVSWMIRILIGFLVLWIGTNSRNTSMAMTCIAVGGITLFLGFTVGA

SEQ ID NO: 15 - DNA, 1029 bp, Yellow fever virus
gatcaaggatgcgccatcaactttggcgtgagcaagggcgaggagctgttcaccggggtggtgcccatcctggtcgagctggacggcgacgtaaacggccacaagttcagcgtgtccggcgagggcgagggcgatgccacctacggcaagctgaccctgaagttcatctgcaccaccggcaagctgcccgtgccctggcccaccctcgtgaccaccctgacctacggcgtgcagtgcttcagccgctaccccgaccacatgaagcagcacgacttcttcaagtccgccatgcccgaaggctacgtccaggagcgcaccatcttcttcaaggacgacggcaactacaagacccgcgccgaggtgaagttcgagggcgacaccctggtgaaccgcatcgagctgaagggcatcgacttcaaggaggacggcaacatcctggggcacaagctggagtacaactacaacagccacaacgtctatatcatggccgacaagcagaagaacggcatcaaggtgaacttcaagatccgccacaacatcgaggacggcagcgtgcagctcgccgaccactaccagcagaacacccccatcggcgacggccccgtgctgctgcccgacaaccactacctgagcacccagtccgccctgagcaaagaccccaacgagaagcgcgatcacatggtcctgctggagttcgtgaccgccgccgggatcactctcggcatggacgagctgtacaagaagatgtttgagtccacatacagaggtgcaaaacgaatggccattctaggtgaaacagcttgggattttggttccgttggtggactgttcacatcattgggaaaggctgtgcaccaggtttttggaagtgtgtatacaaccatgtttggaggagtctcatggatgattagaatcctaattgggttcttagtgttgtggattggcacgaactccaggaacacttcaatggctatgacgtgcatagctgttggaggaatcactctgtttctgggcttcacagttggcgcc

SEQ ID NO: 16 - protein, 343 aa, Yellow fever virus
DQGCAINFGVSKGEELFTGVVPILVELDGDVNGHKFSVSGEGEGDATYGKLTLKFICTTGKLPVPWPTLVTTLTYGVQCFSRYPDHMKQHDFFKSAMPEGYVQERTIFFKDDGNYKTRAEVKFEGDTLVNRIELKGIDFKEDGNILGHKLEYNYNSHNVYIMADKQKNGIKVNFKIRHNIEDGSVQLADHYQQNTPIGDGPVLLPDNHYLSTQSALSKDPNEKRDHMVLLEFVTAAGITLGMDELYKKMFESTYRGAKRMAILGETAWDFGSVGGLFTSLGKAVHQVFGSVYTTMFGGVSWMIRILIGFLVLWIGTNSRNTSMAMTCIAVGGITLFLGFTVGA

SEQ ID NO: 17 - DNA, 1080 bp, Yellow fever virus
gatcaaggatgcgccatcaacttcggccgaaagggatcacaaacctccaacacaactaaatgggctcctcccggacaaggaagtccaggtagcaagggcgaggagctgttcaccggggtggtgcccatcctggtcgagctggacggcgacgtaaacggccacaagttcagcgtgtccggcgagggcgagggcgatgccacctacggcaagctgaccctgaagttcatctgcaccaccggcaagctgcccgtgccctggcccaccctcgtgaccaccctgacctacggcgtgcagtgcttcagccgctaccccgaccacatgaagcagcacgacttcttcaagtccgccatgcccgaaggctacgtccaggagcgcaccatcttcttcaaggacgacggcaactacaagacccgcgccgaggtgaagttcgagggcgacaccctggtgaaccgcatcgagctgaagggcatcgacttcaaggaggacggcaacatcctggggcacaagctggagtacaactacaacagccacaacgtctatatcatggccgacaagcagaagaacggcatcaaggtgaacttcaagatccgccacaacatcgaggacggcagcgtgcagctcgccgaccactaccagcagaacacccccatcggcgacggccccgtgctgctgcccgacaaccactacctgagcacccagtccgccctgagcaaagaccccaacgagaagcgcgatcacatggtcctgctggagttcgtgaccgccgccgggatcactctcggcatggacgagctgtacaagggtagcagtccactgtctcatcgcagtaaaaggagcctatcctgtcggccacccatggtcaaagagggaagctcaataggaacatcattgggaaaggctgtgcaccaggtttttggaagtgtgtatacaaccatgtttggaggagtctcatggatgattagaatcctaattgggttcttagtgttgtggattggcacgaactcaaggaacacttcaatggctatgacgtgcatagctgttggaggaatcactctgtttctgggcttcacagttggcgcc

SEQ ID NO: 18 - protein, 360 aa, Yellow fever virus
DQGCAINFGRKGSQTSNTTKWAPPGQGSPGSKGEELFTGVVPILVELDGDVNGHKFSVSGEGEGDATYGKLTLKFICTTGKLPVPWPTLVTTLTYGVQCFSRYPDHMKQHDFFKSAMPEGYVQERTIFFKDDGNYKTRAEVKFEGDTLVNRIELKGIDFKEDGNILGHKLEYNYNSHNVYIMADKQKNGIKVNFKIRHNIEDGSVQLADHYQQNTPIGDGPVLLPDNHYLSTQSALSKDPNEKRDHMVLLEFVTAAGITLGMDELYKGSSPLSHRSKRSLSCRPPMVKEGSSIGTSLGKAVHQVFGSVYTTMFGGVSWMIRILIGFLVLWIGTNSRNTSMAMTCIAVGGITLFLGFTVGA

SEQ ID NO: 19 - DNA, 1173 bp, Yellow fever virus
gatcaaggatgcgccatcaacttcggccgaaagggatcacaaacctccaacacaactaaatgggctcctcccggacaaggaagtcccgggagcaagggcgaggagctgttcaccggggtggtgcccatcctggtcgagctggacggcgacgtaaacggccacaagttcagcgtgtccggcgagggcgagggcgatgccacctacggcaagctgaccctgaagttcatctgcaccaccggcaagctgcccgtgccctggcccaccctcgtgaccaccctgacctacggcgtgcagtgcttcagccgctaccccgaccacatgaagcagcacgacttcttcaagtccgccatgcccgaaggctacgtccaggagcgcaccatcttcttcaaggacgacggcaactacaagacccgcgccgaggtgaagttcgagggcgacaccctggtgaaccgcatcgagctgaagggcatcgacttcaaggaggacggcaacatcctggggcacaagctggagtacaactacaacagccacaacgtctatatcatggccgacaagcagaagaacggcatcaaggtgaacttcaagatccgccacaacatcgaggacggcagcgtgcagctcgccgaccactaccagcagaacacccccatcggcgacggccccgtgctgctgcccgacaaccactacctgagcacccagtccgccctgagcaaagaccccaacgagaagcgcgatcacatggtcctgctggagttcgtgaccgccgccgggatcactctcggcatggacgagctgtacaagtccggaagcagtccactgtctcatcgcagtaaaaggagcctatcctgtcggccacccatggtcaaagagggaagctcaataggaaagatgtttgagtccacatacagaggtgcaaaacgaatggccattctaggtgaaacagcttgggattttggttccgttggtggactgttcacatcattgggaaaggctgtgcaccaggtttttggaagtgtgtatacaaccatgtttggaggagtctcatggatgattagaatcctaattgggttcttagtgttgtggattggcacgaactccaggaacacttcaatggctatgacgtgcatagctgttggaggaatcactctgtttctgggcttcacagttggcgcc

SEQ ID NO: 20 - protein, 391 aa, Yellow fever virus
DQGCAINFGRKGSQTSNTTKWAPPGQGSPGSKGEELFTGVVPILVELDGDVNGHKFSVSGEGEGDATYGKLTLKFICTTGKLPVPWPTLVTTLTYGVQCFSRYPDHMKQHDFFKSAMPEGYVQERTIFFKDDGNYKTRAEVKFEGDTLVNRIELKGIDFKEDGNILGHKLEYNYNSHNVYIMADKQKNGIKVNFKIRHNIEDGSVQLADHYQQNTPIGDGPVLLPDNHYLSTQSALSKDPNEKRDHMVLLEFVTAAGITLGMDELYKSGSSPLSHRSKRSLSCRPPMVKEGSSIGKMFESTYRGAKRMAILGETAWDFGSVGGLFTSLGKAVHQVFGSVYTTMFGGVSWMIRILIGFLVLWIGTNSRNTSMAMTCIAVGGITLFLGFTVGA

SEQ ID NO: 21 - DNA, 1068 bp, Yellow fever virus
gatcaaggatgcgccatcaacttcggccgaaagtcaggggaagaacatgcagtcggaaatactacaggaagtagcaagggcgaggagctgttcaccggggtggtgcccatcctggtcgagctggacggcgacgtaaacggccacaagttcagcgtgtccggcgagggcgagggcgatgccacctacggcaagctgaccctgaagttcatctgcaccaccggcaagctgcccgtgccctggcccaccctcgtgaccaccctgacctacggcgtgcagtgcttcagccgctaccccgaccacatgaagcagcacgacttcttcaagtccgccatgcccgaaggctacgtccaggagcgcaccatcttcttcaaggacgacggcaactacaagacccgcgccgaggtgaagttcgagggcgacaccctggtgaaccgcatcgagctgaagggcatcgacttcaaggaggacggcaacatcctggggcacaagctggagtacaactacaacagccacaacgtctatatcatggccgacaagcagaagaacggcatcaaggtgaacttcaagatccgccacaacatcgaggacggcagcgtgcagctcgccgaccactaccagcagaacacccccatcggcgacggccccgtgctgctgcccgacaaccactacctgagcacccagtccgccctgagcaaagaccccaacgagaagcgcgatcacatggtcctgctggagttcgtgaccgccgccgggatcactctcggcatggacgagctgtacaagagtggagggaaacaggaaggctcacggacaaggcgctcagtgctgatcccatcccatgctcagggaaaagagggaagctcaataggaacatcattgggaaaggctgtgcaccaggtttttggaagtgtgtatacaaccatgtttggaggagtctcatggatgattagaatcctaattgggttcttagtgttgtggattggcacgaactcaaggaacacttcaatggctatgacgtgcatagctgttggaggaatcactctgtttctgggcttcacagttggcgcc

SEQ ID NO: 22 - protein, 356 aa, Yellow fever virus
DQGCAINFGRKSGEEHAVGNTTGSSKGEELFTGVVPILVELDGDVNGHKFSVSGEGEGDATYGKLTLKFICTTGKLPVPWPTLVTTLTYGVQCFSRYPDHMKQHDFFKSAMPEGYVQERTIFFKDDGNYKTRAEVKFEGDTLVNRIELKGIDFKEDGNILGHKLEYNYNSHNVYIMADKQKNGIKVNFKIRHNIEDGSVQLADHYQQNTPIGDGPVLLPDNHYLSTQSALSKDPNEKRDHMVLLEFVTAAGITLGMDELYKSGGKQEGSRTRRSVLIPSHAQGKEGSSIGTSLGKAVHQVFGSVYTTMFGGVSWMIRILIGFLVLWIGTNSRNTSMAMTCIAVGGITLFLGFTVGA

SEQ ID NO: 23 - DNA, 1185 bp, Yellow fever virus
gatcaaggatgcgccatcaacttcggccgaaagggatcacaaacctccaacacaactaaatgggctcctcccggacaaggaagtcccgggagcaagggcgaggagctgttcaccggggtggtgcccatcctggtcgagctggacggcgacgtaaacggccacaagttcagcgtgtccggcgagggcgagggcgatgccacctacggcaagctgaccctgaagttcatctgcaccaccggcaagctgcccgtgccctggcccaccctcgtgaccaccctgacctacggcgtgcagtgcttcagccgctaccccgaccacatgaagcagcacgacttcttcaagtccgccatgcccgaaggctacgtccaggagcgcaccatcttcttcaaggacgacggcaactacaagacccgcgccgaggtgaagttcgagggcgacaccctggtgaaccgcatcgagctgaagggcatcgacttcaaggaggacggcaacatcctggggcacaagctggagtacaactacaacagccacaacgtctatatcatggccgacaagcagaagaacggcatcaaggtgaacttcaagatccgccacaacatcgaggacggcagcgtgcagctcgccgaccactaccagcagaacacccccatcggcgacggccccgtgctgctgcccgacaaccactacctgagcacccagtccgccctgagcaaagaccccaacgagaagcgcgatcacatggtcctgctggagttcgtgaccgccgccgggatcactctcggcatggacgagctgtacaagtccggaagcagtccacagctgttgaattttgaccttcttaagcttgctggagacgtcgagtccaaccctgggccaaaggagggaagctcaataggaaagatgtttgagtccacatacagaggtgcaaaacgaatggccattctaggtgaaacagcttgggattttggttccgttggtggactgttcacatcattgggaaaggctgtgcaccaggtttttggaagtgtgtatacaaccatgtttggaggagtctcatggatgattagaatcctaattgggttcttagtgttgtggattggcacgaactccaggaacacttcaatggctatgacgtgcatagctgttggaggaatcactctgtttctgggcttcacagttggcgcc

SEQ ID NO: 24 - protein, 395 aa, Yellow fever virus
DQGCAINFGRKGSQTSNTTKWAPPGQGSPGSKGEELFTGVVPILVELDGDVNGHKFSVSGEGEGDATYGKLTLKFICTTGKLPVPWPTLVTTLTYGVQCFSRYPDHMKQHDFFKSAMPEGYVQERTIFFKDDGNYKTRAEVKFEGDTLVNRIELKGIDFKEDGNILGHKLEYNYNSHNVYIMADKQKNGIKVNFKIRHNIEDGSVQLADHYQQNTPIGDGPVLLPDNHYLSTQSALSKDPNEKRDHMVLLEFVTAAGITLGMDELYKSGSSPQLLNFDLLKLAGDVESNPGPKEGSSIGKMFESTYRGAKRMAILGETAWDFGSVGGLFTSLGKAVHQVFGSVYTTMFGGVSWMIRILIGFLVLWIGTNSRNTSMAMTCIAVGGITLFLGFTVGA

SEQ ID NO: 25 - DNA, 711 bp, Aequorea victoria
agcaagggcgaggagctgttcaccggggtggtgcccatcctggtcgagctggacggcgacgtaaacggccacaagttcagcgtgtccggcgagggcgagggcgatgccacctacggcaagctgaccctgaagttcatctgcaccaccggcaagctgcccgtgccctggcccaccctcgtgaccaccctgacctacggcgtgcagtgcttcagccgctaccccgaccacatgaagcagcacgacttcttcaagtccgccatgcccgaaggctacgtccaggagcgcaccatcttcttcaaggacgacggcaactacaagacccgcgccgaggtgaagttcgagggcgacaccctggtgaaccgcatcgagctgaagggcatcgacttcaaggaggacggcaacatcctggggcacaagctggagtacaactacaacagccacaacgtctatatcatggccgacaagcagaagaacggcatcaaggtgaacttcaagatccgccacaacatcgaggacggcagcgtgcagctcgccgaccactaccagcagaacacccccatcggcgacggccccgtgctgctgcccgacaaccactacctgagcacccagtccgccctgagcaaagaccccaacgagaagcgcgatcacatggtcctgctggagttcgtgaccgccgccgggatcactctcggcatggacgagctgtacaag

SEQ ID NO: 26 - protein, 237 aa, Aequorea victoria
SKGEELFTGVVPILVELDGDVNGHKFSVSGEGEGDATYGKLTLKFICTTGKLPVPWPTLVTTLTYGVQCFSRYPDHMKQHDFFKSAMPEGYVQERTIFFKDDGNYKTRAEVKFEGDTLVNRIELKGIDFKEDGNILGHKLEYNYNSHNVYIMADKQKNGIKVNFKIRHNIEDGSVQLADHYQQNTPIGDGPVLLPDNHYLSTQSALSKDPNEKRDHMVLLEFVTAAGITLGMDELYK

SEQ ID NO: 27 - DNA, 27 bp, Yellow fever virus
gatcaaggatgcgccatcaacttcggc

SEQ ID NO: 28 - protein, 9 aa, Yellow fever virus
DQGCAINFG

SEQ ID NO: 29 - DNA, 63 bp, Rabies virus
cgaaagggatcacaaacctccaacacaactaaatgggctcctcccggacaaggaagtcccggg

SEQ ID NO: 30 - protein, 21 aa, Rabies virus
RKGSQTSNTTKWAPPGQGSPG

SEQ ID NO: 31 - DNA, 39 bp, Rabies virus
caaacctccaacacaactaaatgggctcctcccggacaa

SEQ ID NO: 32 - protein, 13 aa, Rabies virus
QTSNTTKWAPPGQ

SEQ ID NO: 33 - DNA, 12 bp, Artificial Sequence
  Spacer 5� of motif bearing the N-glycosylation site for the rabies virus G protein
cgaaagggatca

SEQ ID NO: 34 - protein, 4 aa, Artificial Sequence
  N-terminal spacer of motif bearing the N-glycosylation site for the rabies virus G protein
RKGS

SEQ ID NO: 35 - DNA, 12 bp, Artificial Sequence
  Spacer 3� of motif bearing the N-glycosylation site for the rabies virus G protein
ggaagtcccggg

SEQ ID NO: 36 - protein, 4 aa, Artificial Sequence
  C-terminal spacer of motif bearing the N-glycosylation site for the rabies virus G protein
GSPG

SEQ ID NO: 37 - DNA, 45 bp, Dengue virus type 2
cgaaagtcaggggaagaacatgcagtcggaaatactacaggaagt

SEQ ID NO: 38 - protein, 15 aa, Dengue virus type 2
RKSGEEHAVGNTTGS

SEQ ID NO: 39 - DNA, 33 bp, Dengue virus type 2
tcaggggaagaacatgcagtcggaaatactaca

SEQ ID NO: 40 - protein, 11 aa, Dengue virus type 2
SGEEHAVGNTT

SEQ ID NO: 41 - DNA, 6 bp, Artificial Sequence
  Spacer 5� of motif bearing the N-glycosylation site for the dengue virus 2 E protein
cgaaag

SEQ ID NO: 42 - protein, 2 aa, Artificial Sequence
  N-terminal spacer of motif bearing the N-glycosylation site for he dengue virus 2 E protein
RK

SEQ ID NO: 43 - DNA, 6 bp, Artificial Sequence
  Spacer 3� of motif bearing the N-glycosylation site for the dengue virus 2 E protein
ggaagt

SEQ ID NO: 44 - protein, 2 aa, Artificial Sequence
  C-terminal spacer of motif bearing the N-glycosylation site for the dengue virus 2 E protein
GS

SEQ ID NO: 45 - DNA, 84 bp, Homo sapiens
tccggaagcagtccactgtctcatcgcagtaaaaggagcctatcctgtcggccacccatggtcaaagagggaagctcaatagga

SEQ ID NO: 46 - protein, 28 aa, Homo sapiens
SGSSPLSHRSKRSLSCRPPMVKEGSSIG

SEQ ID NO: 47 - DNA, 57 bp, Homo sapiens
agcagtccactgtctcatcgcagtaaaaggagcctatcctgtcggccacccatggtc

SEQ ID NO: 48 - protein, 19 aa, Homo sapiens
SSPLSHRSKRSLSCRPPMV

SEQ ID NO: 49 - DNA, 6 bp, Artificial Sequence
  Spacer 5� of motif bearing the furin cleavage site for human von Willebran factor
tccgga

SEQ ID NO: 50 - protein, 2 aa, Artificial Sequence
  N-terminal spacer of motif bearing the furin cleavage site for human von Willebran factor
SG

SEQ ID NO: 51 - DNA, 21 bp, Artificial Sequence
  Spacer 3� of motif bearing the furin cleavage site for human von Willebran factor
aaagagggaagctcaatagga

SEQ ID NO: 52 - protein, 7 aa, Artificial Sequence
  C-terminal spacer of motif bearing the furin cleavage site for human von Willebran factor
KEGSSIG

SEQ ID NO: 53 - DNA, 87 bp, Tick-borne encephalitis virus
agtggagggaaacaggaaggctcacggacaaggcgctcagtgctgatcccatcccatgctcagggaaaagagggaagctcaatagga

SEQ ID NO: 54 - protein, 29 aa, Tick-borne encephalitis virus
SGGKQEGSRTRRSVLIPSHAQGKEGSSIG

SEQ ID NO: 55 - DNA, 60 bp, Tick-borne encephalitis virus
gggaaacaggaaggctcacggacaaggcgctcagtgctgatcccatcccatgctcaggga

SEQ ID NO: 56 - protein, 20 aa, Tick-borne encephalitis virus
GKQEGSRTRRSVLIPSHAQG

SEQ ID NO: 57 - DNA, 6 bp, Artificial Sequence
  Spacer 5' of motif bearing the furin cleavage site for the prM protein � TBE virus
agtgga

SEQ ID NO: 58 - protein, 2 aa, Artificial Sequence
  N-terminal spacer of motif bearing the furin cleavage site for the prM protein � TBE virus
SG

SEQ ID NO: 59 - DNA, 21 bp, Artificial Sequence
  Spacer 3' of motif bearing the furin cleavage site for the prM protein � TBE virus
aaagagggaagctcaatagga

SEQ ID NO: 60 - protein, 7 aa, Artificial Sequence
  C-terminal spacer of motif bearing the furin cleavage site for the prM protein � TBE virus
KEGSSIG

SEQ ID NO: 61 - DNA, 96 bp, Foot-and-mouth disease virus
tccggaagcagtccacagctgttgaattttgaccttcttaagcttgctggagacgtcgagtccaaccctgggccaaaggagggaagctcaatagga

SEQ ID NO: 62 - protein, 32 aa, Foot-and-mouth disease virus
SGSSPQLLNFDLLKLAGDVESNPGPKEGSSIG

SEQ ID NO: 63 - DNA, 60 bp, Foot-and-mouth disease virus
cagctgttgaattttgaccttcttaagcttgctggagacgtcgagtccaaccctgggcca

SEQ ID NO: 64 - protein, 20 aa, Foot-and-mouth disease virus
QLLNFDLLKLAGDVESNPGP

SEQ ID NO: 65 - DNA, 15 bp, Foot-and-mouth disease virus
tccggaagcagtcca

SEQ ID NO: 66 - protein, 5 aa, Artificial Sequence
  Spacer 5� of motif bearing peptide 2A of Foot-and-mouth disease virus - DNA
SGSSP

SEQ ID NO: 67 - DNA, 21 bp, Artificial Sequence
  N-terminal spacer of motif bearing peptide 2A of Foot-and-mouth disease virus
aaggagggaagctcaatagga

SEQ ID NO: 68 - protein, 7 aa, Artificial Sequence
  Spacer 3� of motif bearing peptide 2A of Foot-and-mouth disease virus
KEGSSIG

SEQ ID NO: 69 - DNA, 198 bp, Dengue virus type 4
acatcattgggaaaggctgtgcaccaggtttttggaagtgtgtatacaaccatgtttggaggagtctcatggatgattagaatcctaattgggttcttagtgttgtggattggcacgaactcaaggaacacttcaatggctatgacgtgcatagctgttggaggaatcactctgtttctgggcttcacagttggcgcc

SEQ ID NO: 70 - protein, 66 aa, Dengue virus type 4
TSLGKAVHQVFGSVYTTMFGGVSWMIRILIGFLVLWIGTNSRNTSMAMTCIAVGGITLFLGFTVGA

SEQ ID NO: 71 - DNA, 288 bp, Dengue virus type 4
aagatgtttgagtccacatacagaggtgcaaaacgaatggccattctaggtgaaacagcttgggattttggttccgttggtggactgttcacatcattgggaaaggctgtgcaccaggtttttggaagtgtgtatacaaccatgtttggaggagtctcatggatgattagaatcctaattgggttcttagtgttgtggattggcacgaactccaggaacacttcaatggctatgacgtgcatagctgttggaggaatcactctgtttctgggcttcacagttggcgcc

SEQ ID NO: 72 - protein, 96 aa, Dengue virus type 4
KMFESTYRGAKRMAILGETAWDFGSVGGLFTSLGKAVHQVFGSVYTTMFGGVSWMIRILIGFLVLWIGTNSRNTSMAMTCIAVGGITLFLGFTVGA